European Patent Specification EP 3 535 300 B1, published October 22, 2025. Title: ACTIVATABLE ANTI-CTLA-4 ANTIBODIES AND USES THEREOF. Applicant: BRISTOL-MYERS SQUIBB COMPANY. The sequence listing filed with the application follows.

SEQUENCE LISTING (570 sequences)

SEQ ID NO: 1 - protein, 15 aa, Artificial Sequence
  Masking Moiety - YV1
DFSCLHSMYNVCLDP

SEQ ID NO: 2 - protein, 15 aa, Artificial Sequence
  Masking Moiety - YV2
QPCAQMYGYSMCPHT

SEQ ID NO: 3 - protein, 15 aa, Artificial Sequence
  Masking Moiety - YV3
LHCRTQMYGYNLCPY

SEQ ID NO: 4 - protein, 15 aa, Artificial Sequence
  Masking Moiety - YV4
LHCRTQLYGYNLCPY

SEQ ID NO: 5 - protein, 9 aa, Artificial Sequence
  Masking Moiety - YV5
CTYSFFNVC

SEQ ID NO: 6 - protein, 10 aa, Artificial Sequence
  Masking Moiety - YV6
CAQMYGYSMC

SEQ ID NO: 7 - protein, 7 aa, Artificial Sequence
  Masking Moiety - YV7
CPNHPMC

SEQ ID NO: 8 - protein, 15 aa, Artificial Sequence
  Masking Moiety - YV8
GTACTYSFFNVCLDP

SEQ ID NO: 9 - protein, 15 aa, Artificial Sequence
  Masking Moiety - YV9
FGTACPNHPMCHDWQ

SEQ ID NO: 10 - protein, 15 aa, Artificial Sequence
  Masking Moiety - YV10
SACAYWMFGVNLCPY

SEQ ID NO: 11 - protein, 11 aa, Artificial Sequence
  Masking Moiety - YV11
CRTQLYGYNLC

SEQ ID NO: 12 - protein, 11 aa, Artificial Sequence
  Masking Moiety - YV12
CRTQIYGYNLC

SEQ ID NO: 13 - protein, 15 aa, Artificial Sequence
  Masking Moiety - YV13
LHCRTQIYGYNLCPY

SEQ ID NO: 14 - protein, 11 aa, Artificial Sequence
  Masking Moiety - YV14
CPNHPMCHDWQ

SEQ ID NO: 15 - protein, 14 aa, Artificial Sequence
  Masking Moiety - YV15
GTACPNHPMCHDWQ

SEQ ID NO: 16 - protein, 13 aa, Artificial Sequence
  Masking Moiety - YV16
CAYWMFGVNLCPY

SEQ ID NO: 17 - protein, 15 aa, Artificial Sequence
  Masking Moiety - YV17
QECHLYMYGVNLCPY

SEQ ID NO: 18 - protein, 13 aa, Artificial Sequence
  Masking Moiety - YV18
CHLYMYGVNLCPY

SEQ ID NO: 19 - protein, 15 aa, Artificial Sequence
  Masking Moiety - YV19
GQCQFYMFGYNLCPY

SEQ ID NO: 20 - protein, 15 aa, Artificial Sequence
  Masking Moiety - YV20
LSTCMYSFFNVCLDP

SEQ ID NO: 21 - protein, 12 aa, Artificial Sequence
  Masking Moiety - YV21
CLHSMYNVCLDP

SEQ ID NO: 22 - protein, 9 aa, Artificial Sequence
  Masking Moiety - YV22
CLHSMYNVC

SEQ ID NO: 23 - protein, 12 aa, Artificial Sequence
  Masking Moiety - YV23
CLHSLYNVCLDP

SEQ ID NO: 24 - protein, 12 aa, Artificial Sequence
  Masking Moiety - YV24
CLHSAYNVCLDP

SEQ ID NO: 25 - protein, 12 aa, Artificial Sequence
  Masking Moiety - YV25
CMYSFFNVCLDP

SEQ ID NO: 26 - protein, 9 aa, Artificial Sequence
  Masking Moiety - YV26
CMYSFFNVC

SEQ ID NO: 27 - protein, 12 aa, Artificial Sequence
  Masking Moiety - YV27
QPCAQMYGYSMC

SEQ ID NO: 28 - protein, 13 aa, Artificial Sequence
  Masking Moiety - YV28
CAQLYGYSMCPHT

SEQ ID NO: 29 - protein, 13 aa, Artificial Sequence
  Masking Moiety - YV29
CAQMYGYSMCAHT

SEQ ID NO: 30 - protein, 13 aa, Artificial Sequence
  Masking Moiety - YV30
CAQMYGYSMCPAT

SEQ ID NO: 31 - protein, 13 aa, Artificial Sequence
  Masking Moiety - YV31
CAQMYGYSMCPHT

SEQ ID NO: 32 - protein, 11 aa, Artificial Sequence
  Masking Moiety - YV32
CPNHPLCHDWQ

SEQ ID NO: 33 - protein, 11 aa, Artificial Sequence
  Masking Moiety - YV33
CPNHPMCADWQ

SEQ ID NO: 34 - protein, 11 aa, Artificial Sequence
  Masking Moiety - YV34
CPNHPMCHAWQ

SEQ ID NO: 35 - protein, 11 aa, Artificial Sequence
  Masking Moiety - YV35
CPNHPMCHDAQ

SEQ ID NO: 36 - protein, 11 aa, Artificial Sequence
  Masking Moiety - YV36
CPNHPMCHDWA

SEQ ID NO: 37 - protein, 10 aa, Artificial Sequence
  Masking Moiety - YV37
GTACPNHPMC

SEQ ID NO: 38 - protein, 13 aa, Artificial Sequence
  Masking Moiety - YV38
LHCRTQLYGYNLC

SEQ ID NO: 39 - protein, 13 aa, Artificial Sequence
  Masking Moiety - YV39
CRTQLYGYNLCPY

SEQ ID NO: 40 - protein, 13 aa, Artificial Sequence
  Masking Moiety - YV40
CRTQLYGYNLCAY

SEQ ID NO: 41 - protein, 13 aa, Artificial Sequence
  Masking Moiety - YV41
CRTQLYGYNLCPA

SEQ ID NO: 42 - protein, 15 aa, Artificial Sequence
  Masking Moiety - YV42
FGTACPNHPLCHDWQ

SEQ ID NO: 43 - protein, 11 aa, Artificial Sequence
  Masking Moiety - YV43
CPNHPLCHDFQ

SEQ ID NO: 44 - protein, 11 aa, Artificial Sequence
  Masking Moiety - YV44
CPNHPLCHDYQ

SEQ ID NO: 45 - protein, 9 aa, Artificial Sequence
  Masking Moiety - YV45
CPNHPLCPY

SEQ ID NO: 46 - protein, 9 aa, Artificial Sequence
  Masking Moiety - YV46
CPNHPLCPA

SEQ ID NO: 47 - protein, 11 aa, Artificial Sequence
  Masking Moiety - YV47
CMYSFFNVCYP

SEQ ID NO: 48 - protein, 11 aa, Artificial Sequence
  Masking Moiety - YV48
CMYSFFNVCYA

SEQ ID NO: 49 - protein, 11 aa, Artificial Sequence
  Masking Moiety - YV49
CLYSFFNVCYP

SEQ ID NO: 50 - protein, 11 aa, Artificial Sequence
  Masking Moiety - YV50
CLYSFFNVCYA

SEQ ID NO: 51 - protein, 15 aa, Artificial Sequence
  Masking Moiety - YV51
FGAACPNHPICHDWQ

SEQ ID NO: 52 - protein, 15 aa, Artificial Sequence
  Masking Moiety - YV52
FGAACPNHPLCHDWQ

SEQ ID NO: 53 - protein, 15 aa, Artificial Sequence
  Masking Moiety - YV53
FGAACPNHPMCHDAQ

SEQ ID NO: 54 - protein, 12 aa, Artificial Sequence
  Masking Moiety - YV54
CLHSAYNACLDP

SEQ ID NO: 55 - protein, 12 aa, Artificial Sequence
  Masking Moiety - YV55
CAHSAYNVCLDP

SEQ ID NO: 56 - protein, 12 aa, Artificial Sequence
  Masking Moiety - YV56
CLHSAYNVCADP

SEQ ID NO: 57 - protein, 12 aa, Artificial Sequence
  Masking Moiety - YV57
CLHSAYNVCLAP

SEQ ID NO: 58 - protein, 12 aa, Artificial Sequence
  Masking Moiety - YV58
CLHSAYNVCLDA

SEQ ID NO: 59 - protein, 15 aa, Artificial Sequence
  Masking Moiety - YV60
KNTCTYVMYNVCLDP

SEQ ID NO: 60 - protein, 15 aa, Artificial Sequence
  Masking Moiety - YV61
YISDCPYHPMCHDYQ

SEQ ID NO: 61 - protein, 15 aa, Artificial Sequence
  Masking Moiety - YV62
FRNTCPYHPMCHDYR

SEQ ID NO: 62 - protein, 15 aa, Artificial Sequence
  Masking Moiety - YV63
RECHMWMFGVNLCPY

SEQ ID NO: 63 - protein, 15 aa, Artificial Sequence
  Masking Moiety - YV64
AVCHMYMYGYNLCPF

SEQ ID NO: 64 - protein, 15 aa, Artificial Sequence
  Masking Moiety - YV65
RSCPQMYGYSMCPHT

SEQ ID NO: 65 - protein, 15 aa, Artificial Sequence
  Masking Moiety - YV66
QPCAQMFGYSMCPHT

SEQ ID NO: 66 - protein, 15 aa, Artificial Sequence
  Masking Moiety
TAKCTYSFFNVCLDP

SEQ ID NO: 67 - protein, 15 aa, Artificial Sequence
  Masking Moiety
DFSCLYSMYNVCLDP

SEQ ID NO: 68 - protein, 15 aa, Artificial Sequence
  Masking Moiety
DVSCMYMMYNFCLDP

SEQ ID NO: 69 - protein, 7 aa, Artificial Sequence
  Masking Moiety
CPNHPMC

SEQ ID NO: 70 - protein, 11 aa, Artificial Sequence
  Masking Moiety
CMYSFFNVCPY

SEQ ID NO: 71 - protein, 11 aa, Artificial Sequence
  Masking Moiety
CMYSFFNVCPA

SEQ ID NO: 72 - protein, 11 aa, Artificial Sequence
  Masking Moiety
CTYSFFNVCPY

SEQ ID NO: 73 - protein, 11 aa, Artificial Sequence
  Masking Moiety
CTYSFFNVCPA

SEQ ID NO: 74 - protein, 15 aa, Artificial Sequence
  Masking Moiety
GFPCMYSMFNVCLDP

SEQ ID NO: 75 - protein, 15 aa, Artificial Sequence
  Masking Moiety
GLSCMYSMYGYCLDP

SEQ ID NO: 76 - protein, 15 aa, Artificial Sequence
  Masking Moiety
IPCDYWMFGVNLCPY

SEQ ID NO: 77 - protein, 15 aa, Artificial Sequence
  Masking Moiety
QVCHAYMYGYNLCPY

SEQ ID NO: 78 - protein, 15 aa, Artificial Sequence
  Masking Moiety
RMYCTYSFYNVCLDP

SEQ ID NO: 79 - protein, 15 aa, Artificial Sequence
  Masking Moiety
ALSCMYIMYNVCLDP

SEQ ID NO: 80 - protein, 15 aa, Artificial Sequence
  Masking Moiety
DFSCMYVMFNVCLDP

SEQ ID NO: 81 - protein, 15 aa, Artificial Sequence
  Masking Moiety
DFSCVYSMFNVCLDP

SEQ ID NO: 82 - protein, 15 aa, Artificial Sequence
  Masking Moiety
DMNTCPNHPMCYDYR

SEQ ID NO: 83 - protein, 15 aa, Artificial Sequence
  Masking Moiety
DMNTCPRHPMCHDYH

SEQ ID NO: 84 - protein, 15 aa, Artificial Sequence
  Masking Moiety
DSRCMYVMYNVCLDP

SEQ ID NO: 85 - protein, 15 aa, Artificial Sequence
  Masking Moiety
EHLCTYSFYNVCLDP

SEQ ID NO: 86 - protein, 15 aa, Artificial Sequence
  Masking Moiety
ELSCVYSMFGFCLDP

SEQ ID NO: 87 - protein, 15 aa, Artificial Sequence
  Masking Moiety
FTNNCPYHPMCHDYL

SEQ ID NO: 88 - protein, 15 aa, Artificial Sequence
  Masking Moiety
GFSCTYIMYDVCLDP

SEQ ID NO: 89 - protein, 15 aa, Artificial Sequence
  Masking Moiety
GSSCMYSMYNVCLDP

SEQ ID NO: 90 - protein, 15 aa, Artificial Sequence
  Masking Moiety
HFSCMYIMYNVCLDP

SEQ ID NO: 91 - protein, 15 aa, Artificial Sequence
  Masking Moiety
LHCGMWMFGVNLCPK

SEQ ID NO: 92 - protein, 15 aa, Artificial Sequence
  Masking Moiety
LPCQMWMFGHNLCPH

SEQ ID NO: 93 - protein, 15 aa, Artificial Sequence
  Masking Moiety
LPCTMYMYGYNLCPY

SEQ ID NO: 94 - protein, 15 aa, Artificial Sequence
  Masking Moiety
LTCHHWMFGVNLCPY

SEQ ID NO: 95 - protein, 15 aa, Artificial Sequence
  Masking Moiety
NFSCMYSMFNVCLDP

SEQ ID NO: 96 - protein, 15 aa, Artificial Sequence
  Masking Moiety
NNHCMYSFFNICLDP

SEQ ID NO: 97 - protein, 15 aa, Artificial Sequence
  Masking Moiety
NRSCMYIMYNVCLDP

SEQ ID NO: 98 - protein, 15 aa, Artificial Sequence
  Masking Moiety
NSCTMFMFGVNLCPY

SEQ ID NO: 99 - protein, 15 aa, Artificial Sequence
  Masking Moiety
NTCELYMFGVNLCPY

SEQ ID NO: 100 - protein, 15 aa, Artificial Sequence
  Masking Moiety
QHCDMWMFGYNLCPY

SEQ ID NO: 101 - protein, 15 aa, Artificial Sequence
  Masking Moiety
QHCPMYMFGYNLCPF

SEQ ID NO: 102 - protein, 15 aa, Artificial Sequence
  Masking Moiety
QVCHIQMYGFDLCPH

SEQ ID NO: 103 - protein, 15 aa, Artificial Sequence
  Masking Moiety
RACDYWMYGVNLCPY

SEQ ID NO: 104 - protein, 15 aa, Artificial Sequence
  Masking Moiety
RQCHMQMFGYDLCPF

SEQ ID NO: 105 - protein, 15 aa, Artificial Sequence
  Masking Moiety
SGSCLYSFYNVCLDP

SEQ ID NO: 106 - protein, 15 aa, Artificial Sequence
  Masking Moiety
SNGCTYSFFNVCLDP

SEQ ID NO: 107 - protein, 14 aa, Artificial Sequence
  Masking Moiety
STCAQMYGYSMCPH

SEQ ID NO: 108 - protein, 15 aa, Artificial Sequence
  Masking Moiety
SYKCLYSFYNVCLDP

SEQ ID NO: 109 - protein, 15 aa, Artificial Sequence
  Masking Moiety
VLYCTYVMYNVCLDP

SEQ ID NO: 110 - protein, 15 aa, Artificial Sequence
  Masking Moiety
VNCGMWMFGYNLCPK

SEQ ID NO: 111 - protein, 15 aa, Artificial Sequence
  Masking Moiety
YGSCLYSFYNICLDP

SEQ ID NO: 112 - protein, 15 aa, Artificial Sequence
  Masking Moiety
YPCAQMYGYSMCPHT

SEQ ID NO: 113 - protein, 15 aa, Artificial Sequence
  Masking Moiety
AACDLWMFGVNLCPY

SEQ ID NO: 114 - protein, 15 aa, Artificial Sequence
  Masking Moiety
AFCTLAPYNQACIAN

SEQ ID NO: 115 - protein, 15 aa, Artificial Sequence
  Masking Moiety
AGSCLYSMYNVCLDP

SEQ ID NO: 116 - protein, 15 aa, Artificial Sequence
  Masking Moiety
ALCENTMYGYHLCPW

SEQ ID NO: 117 - protein, 15 aa, Artificial Sequence
  Masking Moiety
ALSCMYIMYGVCLDP

SEQ ID NO: 118 - protein, 15 aa, Artificial Sequence
  Masking Moiety
APVCDVLMFGFCMQP

SEQ ID NO: 119 - protein, 15 aa, Artificial Sequence
  Masking Moiety
AQVCSIMMYGTCLMP

SEQ ID NO: 120 - protein, 15 aa, Artificial Sequence
  Masking Moiety
ASTCMYSFYNVCLDP

SEQ ID NO: 121 - protein, 15 aa, Artificial Sequence
  Masking Moiety
AVCEFWMFGFNLCPY

SEQ ID NO: 122 - protein, 15 aa, Artificial Sequence
  Masking Moiety
DANTCPNHPMCYDYH

SEQ ID NO: 123 - protein, 15 aa, Artificial Sequence
  Masking Moiety
DFSCIYIMFDVCLDP

SEQ ID NO: 124 - protein, 15 aa, Artificial Sequence
  Masking Moiety
DFSCMYVMYGFCLDP

SEQ ID NO: 125 - protein, 15 aa, Artificial Sequence
  Masking Moiety
DFTCMYSMYNVCLDP

SEQ ID NO: 126 - protein, 15 aa, Artificial Sequence
  Masking Moiety
DFTCTYSMYNVCLDP

SEQ ID NO: 127 - protein, 15 aa, Artificial Sequence
  Masking Moiety
DHYCTYIMYSICLDP

SEQ ID NO: 128 - protein, 15 aa, Artificial Sequence
  Masking Moiety
DICTNFMFGVNLCPY

SEQ ID NO: 129 - protein, 15 aa, Artificial Sequence
  Masking Moiety
DINTCPYHPMCHDYH

SEQ ID NO: 130 - protein, 15 aa, Artificial Sequence
  Masking Moiety
DKNTCPLHPMCHDYR

SEQ ID NO: 131 - protein, 15 aa, Artificial Sequence
  Masking Moiety
DMNMCPNHPMCHDWH

SEQ ID NO: 132 - protein, 15 aa, Artificial Sequence
  Masking Moiety
DMNSCPNHPMCHDYH

SEQ ID NO: 133 - protein, 15 aa, Artificial Sequence
  Masking Moiety
DMNSCPNHPMCYDYR

SEQ ID NO: 134 - protein, 15 aa, Artificial Sequence
  Masking Moiety
DMNTCPNHPMCFDYR

SEQ ID NO: 135 - protein, 15 aa, Artificial Sequence
  Masking Moiety
DMNTCPNHPMCHDFQ

SEQ ID NO: 136 - protein, 15 aa, Artificial Sequence
  Masking Moiety
DMNTCPNHPMCHDYR

SEQ ID NO: 137 - protein, 15 aa, Artificial Sequence
  Masking Moiety
DMNTCPNHPMCYDYH

SEQ ID NO: 138 - protein, 15 aa, Artificial Sequence
  Masking Moiety
DMNTCPNHPMCYDYK

SEQ ID NO: 139 - protein, 15 aa, Artificial Sequence
  Masking Moiety
DMSTCPNHPMCHDYM

SEQ ID NO: 140 - protein, 15 aa, Artificial Sequence
  Masking Moiety
DRNMCPYHPMCYDYR

SEQ ID NO: 141 - protein, 15 aa, Artificial Sequence
  Masking Moiety
DSCAFMMFGVNLCPY

SEQ ID NO: 142 - protein, 15 aa, Artificial Sequence
  Masking Moiety
DSCRSVFDMVWNCWN

SEQ ID NO: 143 - protein, 15 aa, Artificial Sequence
  Masking Moiety
DTPNCPHHPMCHNHM

SEQ ID NO: 144 - protein, 15 aa, Artificial Sequence
  Masking Moiety
DVSCLYVMYSVCLDP

SEQ ID NO: 145 - protein, 15 aa, Artificial Sequence
  Masking Moiety
DWCASMMFGYNLCPY

SEQ ID NO: 146 - protein, 15 aa, Artificial Sequence
  Masking Moiety
EFSCMYSMFNVCLDP

SEQ ID NO: 147 - protein, 15 aa, Artificial Sequence
  Masking Moiety
EHCDVWMFGFNLCPY

SEQ ID NO: 148 - protein, 15 aa, Artificial Sequence
  Masking Moiety
EPCDYWMFGVNLCPY

SEQ ID NO: 149 - protein, 15 aa, Artificial Sequence
  Masking Moiety
EQCTMWMYGFNLCPY

SEQ ID NO: 150 - protein, 15 aa, Artificial Sequence
  Masking Moiety
ESACSLRMYEVCLQP

SEQ ID NO: 151 - protein, 15 aa, Artificial Sequence
  Masking Moiety
ESCASMYGYSMCPRT

SEQ ID NO: 152 - protein, 15 aa, Artificial Sequence
  Masking Moiety
ESCSYWMFGYNLCPY

SEQ ID NO: 153 - protein, 15 aa, Artificial Sequence
  Masking Moiety
FSNTCPHHPMCYDYR

SEQ ID NO: 154 - protein, 15 aa, Artificial Sequence
  Masking Moiety
FWNTCPHHPMCHDYK

SEQ ID NO: 155 - protein, 15 aa, Artificial Sequence
  Masking Moiety
FYQNCYPPTWCSMFS

SEQ ID NO: 156 - protein, 15 aa, Artificial Sequence
  Masking Moiety
GECSYWMFGYNLCPY

SEQ ID NO: 157 - protein, 15 aa, Artificial Sequence
  Masking Moiety
GGSCMYSFFNICLDP

SEQ ID NO: 158 - protein, 15 aa, Artificial Sequence
  Masking Moiety
GGSCVYVMYNVCLDP

SEQ ID NO: 159 - protein, 15 aa, Artificial Sequence
  Masking Moiety
GHCLMHMYGYNLCPK

SEQ ID NO: 160 - protein, 15 aa, Artificial Sequence
  Masking Moiety
GHCRMSMYEMTLCPR

SEQ ID NO: 161 - protein, 15 aa, Artificial Sequence
  Masking Moiety
GISCVHIMFNFCLDP

SEQ ID NO: 162 - protein, 15 aa, Artificial Sequence
  Masking Moiety
GLCVMYMFGVNLCPY

SEQ ID NO: 163 - protein, 15 aa, Artificial Sequence
  Masking Moiety
GSCDYWMFGYNLCPY

SEQ ID NO: 164 - protein, 15 aa, Artificial Sequence
  Masking Moiety
GSYCMYVMYNVCLDP

SEQ ID NO: 165 - protein, 15 aa, Artificial Sequence
  Masking Moiety
GTKCIYSFYNVCLDP

SEQ ID NO: 166 - protein, 15 aa, Artificial Sequence
  Masking Moiety
GTSTCPYHPMCHDYR

SEQ ID NO: 167 - protein, 15 aa, Artificial Sequence
  Masking Moiety
GTTCTYSFFNVCLDP

SEQ ID NO: 168 - protein, 15 aa, Artificial Sequence
  Masking Moiety
GVCHFFMYGVSMCPA

SEQ ID NO: 169 - protein, 15 aa, Artificial Sequence
  Masking Moiety
GVPCWYSMYNVCLDP

SEQ ID NO: 170 - protein, 15 aa, Artificial Sequence
  Masking Moiety
GVSCMYSMFNICLDP

SEQ ID NO: 171 - protein, 15 aa, Artificial Sequence
  Masking Moiety
HAKCVYSFFNVCLDP

SEQ ID NO: 172 - protein, 15 aa, Artificial Sequence
  Masking Moiety
HDSCMYSMYNFCLDP

SEQ ID NO: 173 - protein, 15 aa, Artificial Sequence
  Masking Moiety
HGNTCPNHPMCHDYQ

SEQ ID NO: 174 - protein, 15 aa, Artificial Sequence
  Masking Moiety
HKGCLYSFYNICLDP

SEQ ID NO: 175 - protein, 15 aa, Artificial Sequence
  Masking Moiety
HKGCLYSFYNVCLDP

SEQ ID NO: 176 - protein, 15 aa, Artificial Sequence
  Masking Moiety
HLSCMYIMYNVCLDP

SEQ ID NO: 177 - protein, 15 aa, Artificial Sequence
  Masking Moiety
HSSCIYSMFNVCLDP

SEQ ID NO: 178 - protein, 15 aa, Artificial Sequence
  Masking Moiety
HTNMCPYHPMCYDYK

SEQ ID NO: 179 - protein, 15 aa, Artificial Sequence
  Masking Moiety
HTPCTYSFFNVCLDP

SEQ ID NO: 180 - protein, 15 aa, Artificial Sequence
  Masking Moiety
IMNTCPYHPMCHDYQ

SEQ ID NO: 181 - protein, 15 aa, Artificial Sequence
  Masking Moiety
IVPCTYMMFGVCLQP

SEQ ID NO: 182 - protein, 15 aa, Artificial Sequence
  Masking Moiety
KKCDYWFYGVNLCPY

SEQ ID NO: 183 - protein, 15 aa, Artificial Sequence
  Masking Moiety
KNTCVYSFFNVCLDP

SEQ ID NO: 184 - protein, 15 aa, Artificial Sequence
  Masking Moiety
KPCAQMYGYSMCPHP

SEQ ID NO: 185 - protein, 15 aa, Artificial Sequence
  Masking Moiety
KPSCMYSFFNVCLDP

SEQ ID NO: 186 - protein, 15 aa, Artificial Sequence
  Masking Moiety
KRPCMYSFYNVCLDP

SEQ ID NO: 187 - protein, 15 aa, Artificial Sequence
  Masking Moiety
KTSCMYSFYNICLDP

SEQ ID NO: 188 - protein, 15 aa, Artificial Sequence
  Masking Moiety
KTTCTYSFFNVCLDP

SEQ ID NO: 189 - protein, 15 aa, Artificial Sequence
  Masking Moiety
LDCQMYWWFGACGDM

SEQ ID NO: 190 - protein, 15 aa, Artificial Sequence
  Masking Moiety
LHCAIYMYGYNLCPF

SEQ ID NO: 191 - protein, 15 aa, Artificial Sequence
  Masking Moiety
LHCPFQMYGYNLCPH

SEQ ID NO: 192 - protein, 15 aa, Artificial Sequence
  Masking Moiety
LHCSMYMYGFNLCPN

SEQ ID NO: 193 - protein, 15 aa, Artificial Sequence
  Masking Moiety
RECMAYMYGYNLCPY

SEQ ID NO: 194 - protein, 15 aa, Artificial Sequence
  Masking Moiety
RHCQMHMFGYDLCPY

SEQ ID NO: 195 - protein, 15 aa, Artificial Sequence
  Masking Moiety
LIHCRYVMYGMCLEP

SEQ ID NO: 196 - protein, 15 aa, Artificial Sequence
  Masking Moiety
LLPCEVMGPSRCKHD

SEQ ID NO: 197 - protein, 15 aa, Artificial Sequence
  Masking Moiety
LPCHAYMYGYSLCPY

SEQ ID NO: 198 - protein, 15 aa, Artificial Sequence
  Masking Moiety
LPCLAYMYGVNLCPN

SEQ ID NO: 199 - protein, 15 aa, Artificial Sequence
  Masking Moiety
LPCMAYMFGFNLCPH

SEQ ID NO: 200 - protein, 15 aa, Artificial Sequence
  Masking Moiety
LPCNFHMFGFNLCPY

SEQ ID NO: 201 - protein, 15 aa, Artificial Sequence
  Masking Moiety
LQCAMYMYGYNLCPY

SEQ ID NO: 202 - protein, 15 aa, Artificial Sequence
  Masking Moiety
LSSCTYSFFNVCLDP

SEQ ID NO: 203 - protein, 15 aa, Artificial Sequence
  Masking Moiety
LTCPFQMYGYNLCPY

SEQ ID NO: 204 - protein, 15 aa, Artificial Sequence
  Masking Moiety
LTSQCSPWYWCQIYD

SEQ ID NO: 205 - protein, 15 aa, Artificial Sequence
  Masking Moiety
LYCPYMMYGYNLCPY

SEQ ID NO: 206 - protein, 15 aa, Artificial Sequence
  Masking Moiety
LYHCTYSFYNVCLDP

SEQ ID NO: 207 - protein, 15 aa, Artificial Sequence
  Masking Moiety
LYRCIYSFYNVCLDP

SEQ ID NO: 208 - protein, 15 aa, Artificial Sequence
  Masking Moiety
MGCSMRMWGMELCPE

SEQ ID NO: 209 - protein, 15 aa, Artificial Sequence
  Masking Moiety
MKCDYWLYGYNLCPY

SEQ ID NO: 210 - protein, 15 aa, Artificial Sequence
  Masking Moiety
MNHCTLHMYNICMDP

SEQ ID NO: 211 - protein, 15 aa, Artificial Sequence
  Masking Moiety
MNPECPHHPMCHNSN

SEQ ID NO: 212 - protein, 15 aa, Artificial Sequence
  Masking Moiety
MPACTYSFFNICLDP

SEQ ID NO: 213 - protein, 15 aa, Artificial Sequence
  Masking Moiety
MPQCHVIMYNLCLDP

SEQ ID NO: 214 - protein, 15 aa, Artificial Sequence
  Masking Moiety
MSTCTYSFFNVCLDP

SEQ ID NO: 215 - protein, 15 aa, Artificial Sequence
  Masking Moiety
MTCNYWFYGVNLCPY

SEQ ID NO: 216 - protein, 15 aa, Artificial Sequence
  Masking Moiety
MYCHQSMFGFRMCPD

SEQ ID NO: 217 - protein, 15 aa, Artificial Sequence
  Masking Moiety
NACAQMYGYSMCPHT

SEQ ID NO: 218 - protein, 15 aa, Artificial Sequence
  Masking Moiety
NDCDISMFDQSLCPY

SEQ ID NO: 219 - protein, 15 aa, Artificial Sequence
  Masking Moiety
NFSCVYVMFNVCLDP

SEQ ID NO: 220 - protein, 15 aa, Artificial Sequence
  Masking Moiety
NFTCALTMYEVCLDP

SEQ ID NO: 221 - protein, 15 aa, Artificial Sequence
  Masking Moiety
NLCHAFMFGFNLCPY

SEQ ID NO: 222 - protein, 15 aa, Artificial Sequence
  Masking Moiety
NLNNCPHHPMCHDYQ

SEQ ID NO: 223 - protein, 15 aa, Artificial Sequence
  Masking Moiety
NPPCMYSFFNICLDP

SEQ ID NO: 224 - protein, 15 aa, Artificial Sequence
  Masking Moiety
NSACTYSFFNVCLDP

SEQ ID NO: 225 - protein, 15 aa, Artificial Sequence
  Masking Moiety
NVCTVSMFGVMLCPS

SEQ ID NO: 226 - protein, 15 aa, Artificial Sequence
  Masking Moiety
PACATLMYSVPLCPA

SEQ ID NO: 227 - protein, 15 aa, Artificial Sequence
  Masking Moiety
PAPCMYSFYNVCLDP

SEQ ID NO: 228 - protein, 15 aa, Artificial Sequence
  Masking Moiety
PLCAEMYGYSMCPHN

SEQ ID NO: 229 - protein, 15 aa, Artificial Sequence
  Masking Moiety
PQCHLYMYGYNLCPY

SEQ ID NO: 230 - protein, 15 aa, Artificial Sequence
  Masking Moiety
PRPCMYSFYNVCLDP

SEQ ID NO: 231 - protein, 15 aa, Artificial Sequence
  Masking Moiety
QHCPFQMYGYNLCPY

SEQ ID NO: 232 - protein, 15 aa, Artificial Sequence
  Masking Moiety
QHCQMHMFGYNLCPY

SEQ ID NO: 233 - protein, 15 aa, Artificial Sequence
  Masking Moiety
QHSCMYSFFNVCLDP

SEQ ID NO: 234 - protein, 15 aa, Artificial Sequence
  Masking Moiety
QKCHSYLYGVNLCPY

SEQ ID NO: 235 - protein, 15 aa, Artificial Sequence
  Masking Moiety
QKCNMFMFGYNLCPY

SEQ ID NO: 236 - protein, 15 aa, Artificial Sequence
  Masking Moiety
QMNDCPNHPMCHDYH

SEQ ID NO: 237 - protein, 15 aa, Artificial Sequence
  Masking Moiety
QPCAQMYGYSMCPAT

SEQ ID NO: 238 - protein, 15 aa, Artificial Sequence
  Masking Moiety
QPCAQMYGYSMCPRT

SEQ ID NO: 239 - protein, 15 aa, Artificial Sequence
  Masking Moiety
RECHFFFYGVNLCPY

SEQ ID NO: 240 - protein, 15 aa, Artificial Sequence
  Masking Moiety
LNCGMFMYGYNLCPY

SEQ ID NO: 241 - protein, 15 aa, Artificial Sequence
  Masking Moiety
RLCTSYMFGYNLCPQ

SEQ ID NO: 242 - protein, 15 aa, Artificial Sequence
  Masking Moiety
RLSCMYSMFNVCLDP

SEQ ID NO: 243 - protein, 15 aa, Artificial Sequence
  Masking Moiety
RNCPFVMFGVNLCPY

SEQ ID NO: 244 - protein, 15 aa, Artificial Sequence
  Masking Moiety
RNGCMYSFFNVCLDP

SEQ ID NO: 245 - protein, 15 aa, Artificial Sequence
  Masking Moiety
RNGCVYSFFNVCLDP

SEQ ID NO: 246 - protein, 15 aa, Artificial Sequence
  Masking Moiety
RPCHLYMFGYNLCPD

SEQ ID NO: 247 - protein, 15 aa, Artificial Sequence
  Masking Moiety
RPCHSYMYGINLCPY

SEQ ID NO: 248 - protein, 15 aa, Artificial Sequence
  Masking Moiety
RSCDMIMFGFNLCPY

SEQ ID NO: 249 - protein, 15 aa, Artificial Sequence
  Masking Moiety
RSCPMWFYGVNLCPY

SEQ ID NO: 250 - protein, 15 aa, Artificial Sequence
  Masking Moiety
RSTVCFYDFCGPWER

SEQ ID NO: 251 - protein, 15 aa, Artificial Sequence
  Masking Moiety
RTCHFYMYGVNLCPY

SEQ ID NO: 252 - protein, 15 aa, Artificial Sequence
  Masking Moiety
RTCSMVMFGVNLCPY

SEQ ID NO: 253 - protein, 15 aa, Artificial Sequence
  Masking Moiety
SGKCTYSFFNVCLDP

SEQ ID NO: 254 - protein, 15 aa, Artificial Sequence
  Masking Moiety
SIVCDLYWEATCLRP

SEQ ID NO: 255 - protein, 15 aa, Artificial Sequence
  Masking Moiety
SLSCTYSFFNICLDP

SEQ ID NO: 256 - protein, 15 aa, Artificial Sequence
  Masking Moiety
SMNTCPYHPMCFDYK

SEQ ID NO: 257 - protein, 15 aa, Artificial Sequence
  Masking Moiety
SQCWMWMYGYNLCPK

SEQ ID NO: 258 - protein, 15 aa, Artificial Sequence
  Masking Moiety
SSSCMYSFFNVCLDP

SEQ ID NO: 259 - protein, 15 aa, Artificial Sequence
  Masking Moiety
STACTYSFYNVCLDP

SEQ ID NO: 260 - protein, 15 aa, Artificial Sequence
  Masking Moiety
STCAQMYGYSMCPHT

SEQ ID NO: 261 - protein, 15 aa, Artificial Sequence
  Masking Moiety
STRCVYSFYNVCLDP

SEQ ID NO: 262 - protein, 15 aa, Artificial Sequence
  Masking Moiety
TACGAWMFGVNLCPY

SEQ ID NO: 263 - protein, 15 aa, Artificial Sequence
  Masking Moiety
TGACMYSFYNVCLDP

SEQ ID NO: 264 - protein, 15 aa, Artificial Sequence
  Masking Moiety
TLSCMYSMYNVCLDP

SEQ ID NO: 265 - protein, 15 aa, Artificial Sequence
  Masking Moiety
TSCTVTMYQISMCPY

SEQ ID NO: 266 - protein, 15 aa, Artificial Sequence
  Masking Moiety
VGGCRHSFYNVCLDP

SEQ ID NO: 267 - protein, 15 aa, Artificial Sequence
  Masking Moiety
VHCQMYMYGYNLCPY

SEQ ID NO: 268 - protein, 15 aa, Artificial Sequence
  Masking Moiety
VHNCMYSFFNVCLDP

SEQ ID NO: 269 - protein, 15 aa, Artificial Sequence
  Masking Moiety
VMCKLHMYGIPVCPK

SEQ ID NO: 270 - protein, 15 aa, Artificial Sequence
  Masking Moiety
VNFCNYSMYGICLLP

SEQ ID NO: 271 - protein, 15 aa, Artificial Sequence
  Masking Moiety
VNFCYACYCMSCVFS

SEQ ID NO: 272 - protein, 15 aa, Artificial Sequence
  Masking Moiety
VNQCTYSFFNVCLDP

SEQ ID NO: 273 - protein, 15 aa, Artificial Sequence
  Masking Moiety
VPCPFHMFGYNLCPY

SEQ ID NO: 274 - protein, 15 aa, Artificial Sequence
  Masking Moiety
VRCQMWMYGFNLCPH

SEQ ID NO: 275 - protein, 15 aa, Artificial Sequence
  Masking Moiety
VRPCTYSFFNVCLDP

SEQ ID NO: 276 - protein, 15 aa, Artificial Sequence
  Masking Moiety
VSGCTYSFFNICLDP

SEQ ID NO: 277 - protein, 15 aa, Artificial Sequence
  Masking Moiety
YCSSWDTMTIPACNN

SEQ ID NO: 278 - protein, 15 aa, Artificial Sequence
  Masking Moiety
YDCDLSMFGIEMCPQ

SEQ ID NO: 279 - protein, 15 aa, Artificial Sequence
  Masking Moiety
YGNTCPFHPMCHDYK

SEQ ID NO: 280 - protein, 15 aa, Artificial Sequence
  Masking Moiety
YGYCMYSFFNVCLDP

SEQ ID NO: 281 - protein, 15 aa, Artificial Sequence
  Masking Moiety
YHCTMHMFGYNLCPF

SEQ ID NO: 282 - protein, 15 aa, Artificial Sequence
  Masking Moiety
YMNTCPNHPMCFDYQ

SEQ ID NO: 283 - protein, 15 aa, Artificial Sequence
  Masking Moiety
YMNTCPYHPMCHDYL

SEQ ID NO: 284 - protein, 15 aa, Artificial Sequence
  Masking Moiety
YMNTCPYHPMCHDYR

SEQ ID NO: 285 - protein, 15 aa, Artificial Sequence
  Masking Moiety
YNNCTYSFFNVCLDP

SEQ ID NO: 286 - protein, 15 aa, Artificial Sequence
  Masking Moiety
YPGCQYSFFNVCLDP

SEQ ID NO: 287 - protein, 15 aa, Artificial Sequence
  Masking Moiety
YRSCTHIMYNVCLDP

SEQ ID NO: 288 - protein, 15 aa, Artificial Sequence
  Masking Moiety
YSFCDMLMYDVCLVP

SEQ ID NO: 289 - protein, 15 aa, Artificial Sequence
  Masking Moiety
YSIDCGLSWWCGGMT

SEQ ID NO: 290 - protein, 15 aa, Artificial Sequence
  Masking Moiety
YSTTCPYHPMCHDYH

SEQ ID NO: 291 - protein, 15 aa, Artificial Sequence
  Masking Moiety
YVNTCPHHPMCHDYH

SEQ ID NO: 292 - protein, 15 aa, Artificial Sequence
  Masking Moiety
YVNTCPYHPMCHDYN

SEQ ID NO: 293 - protein, 15 aa, Artificial Sequence
  Masking Moiety - MY03
MCLPPLFELASTCPY

SEQ ID NO: 294 - protein, 15 aa, Artificial Sequence
  Masking Moiety - MY11
LPDCGMWGISCGGTV

SEQ ID NO: 295 - protein, 15 aa, Artificial Sequence
  Masking Moiety - MY16
RDHTCNPRNCHPNMF

SEQ ID NO: 296 - protein, 15 aa, Artificial Sequence
  Masking Moiety - MY04
WRCMPPTWETTQCHT

SEQ ID NO: 297 - protein, 13 aa, Artificial Sequence
  Cleavable Moiety - 2001
ISSGLLSGRSDNH

SEQ ID NO: 298 - protein, 15 aa, Artificial Sequence
  Cleavable Moiety - 2003
ISSGLLSGRSANPRG

SEQ ID NO: 299 - protein, 17 aa, Artificial Sequence
  Cleavable Moiety - 2005
AVGLLAPPSGRSANPRG

SEQ ID NO: 300 - protein, 13 aa, Artificial Sequence
  Cleavable Moiety - 2006
ISSGLLSGRSDDH

SEQ ID NO: 301 - protein, 13 aa, Artificial Sequence
  Cleavable Moiety - 2007
ISSGLLSGRSDIH

SEQ ID NO: 302 - protein, 13 aa, Artificial Sequence
  Cleavable Moiety - 2008
ISSGLLSGRSDQH

SEQ ID NO: 303 - protein, 13 aa, Artificial Sequence
  Cleavable Moiety - 2009
ISSGLLSGRSDTH

SEQ ID NO: 304 - protein, 13 aa, Artificial Sequence
  Cleavable Moiety - 2011
ISSGLLSGRSDNP

SEQ ID NO: 305 - protein, 13 aa, Artificial Sequence
  Cleavable Moiety - 2012
ISSGLLSGRSANP

SEQ ID NO: 306 - protein, 18 aa, Artificial Sequence
  Cleavable Moiety - 3001
AVGLLAPPGGLSGRSDNH

SEQ ID NO: 307 - protein, 18 aa, Artificial Sequence
  Cleavable Moiety - 3006
AVGLLAPPGGLSGRSDDH

SEQ ID NO: 308 - protein, 18 aa, Artificial Sequence
  Cleavable Moiety - 3007
AVGLLAPPGGLSGRSDIH

SEQ ID NO: 309 - protein, 18 aa, Artificial Sequence
  Cleavable Moiety - 3008
AVGLLAPPGGLSGRSDQH

SEQ ID NO: 310 - protein, 18 aa, Artificial Sequence
  Cleavable Moiety - 3009
AVGLLAPPGGLSGRSDTH

SEQ ID NO: 311 - protein, 18 aa, Artificial Sequence
  Cleavable Moiety - 3011
AVGLLAPPGGLSGRSDNP

SEQ ID NO: 312 - protein, 18 aa, Artificial Sequence
  Cleavable Moiety - 3012
AVGLLAPPGGLSGRSANP

SEQ ID NO: 313 - protein, 8 aa, Artificial Sequence
  Cleavable Moiety
LSGRSDNH

SEQ ID NO: 314 - protein, 10 aa, Artificial Sequence
  Cleavable Moiety
LSGRSANPRG

SEQ ID NO: 315 - protein, 8 aa, Artificial Sequence
  Cleavable Moiety
TGRGPSWV

SEQ ID NO: 316 - protein, 8 aa, Artificial Sequence
  Cleavable Moiety
PLTGRSGG

SEQ ID NO: 317 - protein, 8 aa, Artificial Sequence
  Cleavable Moiety
TARGPSFK

SEQ ID NO: 318 - protein, 12 aa, Artificial Sequence
  Cleavable Moiety
NTLSGRSENHSG

SEQ ID NO: 319 - protein, 12 aa, Artificial Sequence
  Cleavable Moiety
NTLSGRSGNHGS

SEQ ID NO: 320 - protein, 12 aa, Artificial Sequence
  Cleavable Moiety
TSTSGRSANPRG

SEQ ID NO: 321 - protein, 8 aa, Artificial Sequence
  Cleavable Moiety
TSGRSANP

SEQ ID NO: 322 - protein, 10 aa, Artificial Sequence
  Cleavable Moiety
VHMPLGFLGP

SEQ ID NO: 323 - protein, 8 aa, Artificial Sequence
  Cleavable Moiety
AVGLLAPP

SEQ ID NO: 324 - protein, 8 aa, Artificial Sequence
  Cleavable Moiety
AQNLLGMV

SEQ ID NO: 325 - protein, 8 aa, Artificial Sequence
  Cleavable Moiety
QNQALRMA

SEQ ID NO: 326 - protein, 8 aa, Artificial Sequence
  Cleavable Moiety
LAAPLGLL

SEQ ID NO: 327 - protein, 8 aa, Artificial Sequence
  Cleavable Moiety
STFPFGMF

SEQ ID NO: 328 - protein, 8 aa, Artificial Sequence
  Cleavable Moiety
ISSGLLSS

SEQ ID NO: 329 - protein, 8 aa, Artificial Sequence
  Cleavable Moiety
PAGLWLDP

SEQ ID NO: 330 - protein, 8 aa, Artificial Sequence
  Cleavable Moiety
VAGRSMRP

SEQ ID NO: 331 - protein, 8 aa, Artificial Sequence
  Cleavable Moiety
VVPEGRRS

SEQ ID NO: 332 - protein, 8 aa, Artificial Sequence
  Cleavable Moiety
ILPRSPAF

SEQ ID NO: 333 - protein, 8 aa, Artificial Sequence
  Cleavable Moiety
MVLGRSLL

SEQ ID NO: 334 - protein, 8 aa, Artificial Sequence
  Cleavable Moiety
VAGRSMRP

SEQ ID NO: 335 - protein, 8 aa, Artificial Sequence
  Cleavable Moiety
QGRAITFI

SEQ ID NO: 336 - protein, 8 aa, Artificial Sequence
  Cleavable Moiety
SPRSIMLA

SEQ ID NO: 337 - protein, 8 aa, Artificial Sequence
  Cleavable Moiety
SMLRSMPL

SEQ ID NO: 338 - protein, 18 aa, Artificial Sequence
  Cleavable Moiety
AVGLLAPPGGLSGRSDYH

SEQ ID NO: 339 - protein, 18 aa, Artificial Sequence
  Cleavable Moiety
AVGLLAPPGGLSGRSANI

SEQ ID NO: 340 - protein, 18 aa, Artificial Sequence
  Cleavable Moiety
AVGLLAPPGGLSGRSDNI

SEQ ID NO: 341 - protein, 13 aa, Artificial Sequence
  Cleavable Moiety
ISSGLLSGRSDYH

SEQ ID NO: 342 - protein, 13 aa, Artificial Sequence
  Cleavable Moiety
ISSGLLSGRSANI

SEQ ID NO: 343 - protein, 13 aa, Artificial Sequence
  Cleavable Moiety
ISSGLLSGRSDNI

SEQ ID NO: 344 - protein, 108 aa, Artificial Sequence
  Ipilimumab-VL
EIVLTQSPGTLSLSPGERATLSCRASQSVGSSYLAWYQQKPGQAPRLLIYGAFSRATGIPDRFSGSGSGTDFTLTISRLEPEDFAVYYCQQYGSSPWTFGQGTKVEIK

SEQ ID NO: 345 - protein, 118 aa, Artificial Sequence
  Ipilimumab-VH
QVQLVESGGGVVQPGRSLRLSCAASGFTFSSYTMHWVRQAPGKGLEWVTFISYDGNNKYYADSVKGRFTISRDNSKNTLYLQMNSLRAEDTAIYYCARTGWLGPFDYWGQGTLVTVSS

SEQ ID NO: 346 - protein, 107 aa, Artificial Sequence [sequence omitted]

SEQ ID NO: 347 - protein, 107 aa, Artificial Sequence
  Mouse Kappa constant LC
RADAAPTVSIFPPSSEQLTSGGASVVCFLNNFYPKDINVKWKIDGSERQNGVLNSWTDQDSKDSTYSMSSTLTLTKDEYERHNSYTCEATHKTSTSPIVKSFNRNEC

SEQ ID NO: 348 - protein, 215 aa, Artificial Sequence
  Ipilimumab-Human Kappa LC
EIVLTQSPGTLSLSPGERATLSCRASQSVGSSYLAWYQQKPGQAPRLLIYGAFSRATGIPDRFSGSGSGTDFTLTISRLEPEDFAVYYCQQYGSSPWTFGQGTKVEIKRTVAAPSVFIFPPSDEQLKSGTASVVCLLNNFYPREAKVQWKVDNALQSGNSQESVTEQDSKDSTYSLSSTLTLSKADYEKHKVYACEVTHQGLSSPVTKSFNRGEC

SEQ ID NO: 349 - protein, 215 aa, Artificial Sequence
  Ipilimumab-Mouse Kappa LC
EIVLTQSPGTLSLSPGERATLSCRASQSVGSSYLAWYQQKPGQAPRLLIYGAFSRATGIPDRFSGSGSGTDFTLTISRLEPEDFAVYYCQQYGSSPWTFGQGTKVEIKRADAAPTVSIFPPSSEQLTSGGASVVCFLNNFYPKDINVKWKIDGSERQNGVLNSWTDQDSKDSTYSMSSTLTLTKDEYERHNSYTCEATHKTSTSPIVKSFNRNEC

SEQ ID NO: 350 - protein, 329 aa, Artificial Sequence
  Human IgG1 constant HC
ASTKGPSVFPLAPSSKSTSGGTAALGCLVKDYFPEPVTVSWNSGALTSGVHTFPAVLQSSGLYSLSSVVTVPSSSLGTQTYICNVNHKPSNTKVDKRVEPKSCDKTHTCPPCPAPELLGGPSVFLFPPKPKDTLMISRTPEVTCVVVDVSHEDPEVKFNWYVDGVEVHNAKTKPREEQYNSTYRVVSVLTVLHQDWLNGKEYKCKVSNKALPAPIEKTISKAKGQPREPQVYTLPPSRDELTKNQVSLTCLVKGFYPSDIAVEWESNGQPENNYKTTPPVLDSDGSFFLYSKLTVDKSRWQQGNVFSCSVMHEALHNHYTQKSLSLSPG

SEQ ID NO: 351 - protein, 329 aa, Artificial Sequence
  Mouse IgG1 constant HC
ASTKGPSVFPLAPSSKSTSGGTAALGCLVKDYFPEPVTVSWNSGALTSGVHTFPAVLQSSGLYSLSSVVTVPSSSLGTQTYICNVNHKPSNTKVDKKVEPKSCDKTHTCPPCPAPELLGGPSVFLFPPKPKDTLMISRTPEVTCVVVDVSHEDPEVKFNWYVDGVEVHNAKTKPREEQYASTYRVVSVLTVLHQDWLNGKEYKCKVSNKALPAPIEKTISKAKGQPREPQVYTLPPSREEMTKNQVSLTCLVKGFYPSDIAVEWESNGQPENNYKTTPPVLDSDGSFFLYSKLTVDKSRWQQGNVFSCSVMHEALHNHYTQKSLSLSPG

SEQ ID NO: 352 - protein, 330 aa, Artificial Sequence
  Mouse IgG2a constant HC
AKTTAPSVYPLAPVCGDTTGSSVTLGCLVKGYFPEPVTLTWNSGSLSSGVHTFPAVLQSDLYTLSSSVTVTSSTWPSQSITCNVAHPASSTKVDKKIEPRGPTIKPCPPCKCPAPNLLGGPSVFIFPPKIKDVLMISLSPIVTCVVVDVSEDDPDVQISWFVNNVEVHTAQTQTHREDYNSTLRVVSALPIQHQDWMSGKEFKCKVNNKDLPAPIERTISKPKGSVRAPQVYVLPPPEEEMTKKQVTLTCMVTDFMPEDIYVEWTNNGKTELNYKNTEPVLDSDGSYFMYSKLRVEKKNWVERNSYSCSVVHEGLHNHHTTKSFSRTPGK

SEQ ID NO: 353 - protein, 447 aa, Artificial Sequence
  Ipilimumab-VH-Human IgG1 constant HC
QVQLVESGGGVVQPGRSLRLSCAASGFTFSSYTMHWVRQAPGKGLEWVTFISYDGNNKYYADSVKGRFTISRDNSKNTLYLQMNSLRAEDTAIYYCARTGWLGPFDYWGQGTLVTVSSASTKGPSVFPLAPSSKSTSGGTAALGCLVKDYFPEPVTVSWNSGALTSGVHTFPAVLQSSGLYSLSSVVTVPSSSLGTQTYICNVNHKPSNTKVDKRVEPKSCDKTHTCPPCPAPELLGGPSVFLFPPKPKDTLMISRTPEVTCVVVDVSHEDPEVKFNWYVDGVEVHNAKTKPREEQYNSTYRVVSVLTVLHQDWLNGKEYKCKVSNKALPAPIEKTISKAKGQPREPQVYTLPPSRDELTKNQVSLTCLVKGFYPSDIAVEWESNGQPENNYKTTPPVLDSDGSFFLYSKLTVDKSRWQQGNVFSCSVMHEALHNHYTQKSLSLSPG

SEQ ID NO: 354 - protein, 447 aa, Artificial Sequence
  Ipilimumab-VH-Mouse IgG1 constant HC
QVQLVESGGGVVQPGRSLRLSCAASGFTFSSYTMHWVRQAPGKGLEWVTFISYDGNNKYYADSVKGRFTISRDNSKNTLYLQMNSLRAEDTAIYYCARTGWLGPFDYWGQGTLVTVSSASTKGPSVFPLAPSSKSTSGGTAALGCLVKDYFPEPVTVSWNSGALTSGVHTFPAVLQSSGLYSLSSVVTVPSSSLGTQTYICNVNHKPSNTKVDKKVEPKSCDKTHTCPPCPAPELLGGPSVFLFPPKPKDTLMISRTPEVTCVVVDVSHEDPEVKFNWYVDGVEVHNAKTKPREEQYASTYRVVSVLTVLHQDWLNGKEYKCKVSNKALPAPIEKTISKAKGQPREPQVYTLPPSREEMTKNQVSLTCLVKGFYPSDIAVEWESNGQPENNYKTTPPVLDSDGSFFLYSKLTVDKSRWQQGNVFSCSVMHEALHNHYTQKSLSLSPG

SEQ ID NO: 355 - protein, 448 aa, Artificial Sequence
  Ipilimumab-VH-Mouse IgG2a constant HC
QVQLVESGGGVVQPGRSLRLSCAASGFTFSSYTMHWVRQAPGKGLEWVTFISYDGNNKYYADSVKGRFTISRDNSKNTLYLQMNSLRAEDTAIYYCARTGWLGPFDYWGQGTLVTVSSAKTTAPSVYPLAPVCGDTTGSSVTLGCLVKGYFPEPVTLTWNSGSLSSGVHTFPAVLQSDLYTLSSSVTVTSSTWPSQSITCNVAHPASSTKVDKKIEPRGPTIKPCPPCKCPAPNLLGGPSVFIFPPKIKDVLMISLSPIVTCVVVDVSEDDPDVQISWFVNNVEVHTAQTQTHREDYNSTLRVVSALPIQHQDWMSGKEFKCKVNNKDLPAPIERTISKPKGSVRAPQVYVLPPPEEEMTKKQVTLTCMVTDFMPEDIYVEWTNNGKTELNYKNTEPVLDSDGSYFMYSKLRVEKKNWVERNSYSCSVVHEGLHNHHTTKSFSRTPGK

SEQ ID NO: 356 - protein, 262 aa, Artificial Sequence
  Spacer - YV01-2001  LC
QGQSGQGDFSCLHSMYNVCLDPGGGSSGGSISSGLLSGRSDNHGGGSEIVLTQSPGTLSLSPGERATLSCRASQSVGSSYLAWYQQKPGQAPRLLIYGAFSRATGIPDRFSGSGSGTDFTLTISRLEPEDFAVYYCQQYGSSPWTFGQGTKVEIKRTVAAPSVFIFPPSDEQLKSGTASVVCLLNNFYPREAKVQWKVDNALQSGNSQESVTEQDSKDSTYSLSSTLTLSKADYEKHKVYACEVTHQGLSSPVTKSFNRGEC

SEQ ID NO: 357 - protein, 255 aa, Artificial Sequence
  YV01-2001 LC
DFSCLHSMYNVCLDPGGGSSGGSISSGLLSGRSDNHGGGSEIVLTQSPGTLSLSPGERATLSCRASQSVGSSYLAWYQQKPGQAPRLLIYGAFSRATGIPDRFSGSGSGTDFTLTISRLEPEDFAVYYCQQYGSSPWTFGQGTKVEIKRTVAAPSVFIFPPSDEQLKSGTASVVCLLNNFYPREAKVQWKVDNALQSGNSQESVTEQDSKDSTYSLSSTLTLSKADYEKHKVYACEVTHQGLSSPVTKSFNRGEC

SEQ ID NO: 358 - protein, 262 aa, Artificial Sequence
  Spacer - YV02-2001 LC
QGQSGQGQPCAQMYGYSMCPHTGGGSSGGSISSGLLSGRSDNHGGGSEIVLTQSPGTLSLSPGERATLSCRASQSVGSSYLAWYQQKPGQAPRLLIYGAFSRATGIPDRFSGSGSGTDFTLTISRLEPEDFAVYYCQQYGSSPWTFGQGTKVEIKRTVAAPSVFIFPPSDEQLKSGTASVVCLLNNFYPREAKVQWKVDNALQSGNSQESVTEQDSKDSTYSLSSTLTLSKADYEKHKVYACEVTHQGLSSPVTKSFNRGEC

SEQ ID NO: 359 - protein, 255 aa, Artificial Sequence
  YV02-2001 LC
QPCAQMYGYSMCPHTGGGSSGGSISSGLLSGRSDNHGGGSEIVLTQSPGTLSLSPGERATLSCRASQSVGSSYLAWYQQKPGQAPRLLIYGAFSRATGIPDRFSGSGSGTDFTLTISRLEPEDFAVYYCQQYGSSPWTFGQGTKVEIKRTVAAPSVFIFPPSDEQLKSGTASVVCLLNNFYPREAKVQWKVDNALQSGNSQESVTEQDSKDSTYSLSSTLTLSKADYEKHKVYACEVTHQGLSSPVTKSFNRGEC

SEQ ID NO: 360 - protein, 262 aa, Artificial Sequence
  Spacer - YV03-2001 LC
QGQSGQGLHCRTQMYGYNLCPYGGGSSGGSISSGLLSGRSDNHGGGSEIVLTQSPGTLSLSPGERATLSCRASQSVGSSYLAWYQQKPGQAPRLLIYGAFSRATGIPDRFSGSGSGTDFTLTISRLEPEDFAVYYCQQYGSSPWTFGQGTKVEIKRTVAAPSVFIFPPSDEQLKSGTASVVCLLNNFYPREAKVQWKVDNALQSGNSQESVTEQDSKDSTYSLSSTLTLSKADYEKHKVYACEVTHQGLSSPVTKSFNRGEC

SEQ ID NO: 361 - protein, 255 aa, Artificial Sequence
  YV03-2001 LC
LHCRTQMYGYNLCPYGGGSSGGSISSGLLSGRSDNHGGGSEIVLTQSPGTLSLSPGERATLSCRASQSVGSSYLAWYQQKPGQAPRLLIYGAFSRATGIPDRFSGSGSGTDFTLTISRLEPEDFAVYYCQQYGSSPWTFGQGTKVEIKRTVAAPSVFIFPPSDEQLKSGTASVVCLLNNFYPREAKVQWKVDNALQSGNSQESVTEQDSKDSTYSLSSTLTLSKADYEKHKVYACEVTHQGLSSPVTKSFNRGEC

SEQ ID NO: 362 - protein, 261 aa, Artificial Sequence
  Spacer - YV04-2001 LC
QGQSGSLHCRTQLYGYNLCPYGGGSSGGSISSGLLSGRSDNHGGGSEIVLTQSPGTLSLSPGERATLSCRASQSVGSSYLAWYQQKPGQAPRLLIYGAFSRATGIPDRFSGSGSGTDFTLTISRLEPEDFAVYYCQQYGSSPWTFGQGTKVEIKRTVAAPSVFIFPPSDEQLKSGTASVVCLLNNFYPREAKVQWKVDNALQSGNSQESVTEQDSKDSTYSLSSTLTLSKADYEKHKVYACEVTHQGLSSPVTKSFNRGEC

SEQ ID NO: 363 - protein, 255 aa, Artificial Sequence
  YV04-2001 LC
LHCRTQLYGYNLCPYGGGSSGGSISSGLLSGRSDNHGGGSEIVLTQSPGTLSLSPGERATLSCRASQSVGSSYLAWYQQKPGQAPRLLIYGAFSRATGIPDRFSGSGSGTDFTLTISRLEPEDFAVYYCQQYGSSPWTFGQGTKVEIKRTVAAPSVFIFPPSDEQLKSGTASVVCLLNNFYPREAKVQWKVDNALQSGNSQESVTEQDSKDSTYSLSSTLTLSKADYEKHKVYACEVTHQGLSSPVTKSFNRGEC

SEQ ID NO: 364 - protein, 256 aa, Artificial Sequence
  Spacer - YV06-2001 LC
QGQSGSCAQMYGYSMCGGGSSGGSISSGLLSGRSDNHGGGSEIVLTQSPGTLSLSPGERATLSCRASQSVGSSYLAWYQQKPGQAPRLLIYGAFSRATGIPDRFSGSGSGTDFTLTISRLEPEDFAVYYCQQYGSSPWTFGQGTKVEIKRTVAAPSVFIFPPSDEQLKSGTASVVCLLNNFYPREAKVQWKVDNALQSGNSQESVTEQDSKDSTYSLSSTLTLSKADYEKHKVYACEVTHQGLSSPVTKSFNRGEC

SEQ ID NO: 365 - protein, 252 aa, Artificial Sequence
  YV06-2001 LC
CAQMYGYSMCGGGSSGGSISSGLLSGRSDNHGGGSEIVLTQSPGTLSLSPGERATLSCRASQSVGSSYLAWYQQKPGQAPRLLIYGAFSRATGIPDRFSGSGYVSGTDFTLTISRLEPEDFAVYYCQQYGSSPWTFGQGTKVEIKRTVAAPSVFIFPPSDEQLKSGTASVVCLLNNFYPREAKVQWKVDNALQSGNSQESVTEQDSKDSTYSLSSTLTLSKADYEKHKVYACEVTHQGLSSPVTKSFNRGEC

SEQ ID NO: 366 - protein, 263 aa, Artificial Sequence
  Spacer - YV09-2001 LC
QGQSGSFGYVTACPNHPMCHDWQGGGSSGGSISSGLLSGRSDNHGGGSEIVLTQSPGTLSLSPGERATLSCRASQSVGSSYLAWYQQKPGQAPRLLIYGAFSRATGIPDRFSGSGSGTDFTLTISRLEPEDFAVYYCQQYGSSPWTFGQGTKVEIKRTVAAPSVFIFPPSDEQLKSGTASVVCLLNNFYPREAKVQWKVDNALQSGNSQESVTEQDSKDSTYSLSSTLTLSKADYEKHKVYACEVTHQGLSSPVTKSFNRGEC

SEQ ID NO: 367 - protein, 255 aa, Artificial Sequence
  YV09-2001 LC
FGTACPNHPMCHDWQGGGSSGGSISSGLLSGRSDNHGGGSEIVLTQSPGTLSLSPGERATLSCRASQSVGSSYLAWYQQKPGQAPRLLIYGAFSRATGIPDRFSGSGSGTDFTLTISRLEPEDFAVYYCQQYGSSPWTFGQGTKVEIKRTVAAPSVFIFPPSDEQLKSGTASVVCLLNNFYPREAKVQWKVDNALQSGNSQESVTEQDSKDSTYSLSSTLTLSKADYEKHKVYACEVTHQGLSSPVTKSFNRGEC

SEQ ID NO: 368 - protein, 258 aa, Artificial Sequence
  Spacer - YV23-2001 LC
QGQSGSCLHSLYNVCLDPGGGSSGGSISSGLLSGRSDNHGGGSEIVLTQSPGTLSLSPGERATLSCRASQSVGSSYLAWYQQKPGQAPRLLIYGAFSRATGIPDRFSGSGSGTDFTLTISRLEPEDFAVYYCQQYGSSPWTFGQGTKVEIKRTVAAPSVFIFPPSDEQLKSGTASVVCLLNNFYPREAKVQWKVDNALQSGNSQESVTEQDSKDSTYSLSSTLTLSKADYEKHKVYACEVTHQGLSSPVTKSFNRGEC

SEQ ID NO: 369 - protein, 252 aa, Artificial Sequence
  YV23-2001 LC
CLHSLYNVCLDPGGGSSGGSISSGLLSGRSDNHGGGSEIVLTQSPGTLSLSPGERATLSCRASQSVGSSYLAWYQQKPGQAPRLLIYGAFSRATGIPDRFSGSGSGTDFTLTISRLEPEDFAVYYCQQYGSSPWTFGQGTKVEIKRTVAAPSVFIFPPSDEQLKSGTASVVCLLNNFYPREAKVQWKVDNALQSGNSQESVTEQDSKDSTYSLSSTLTLSKADYEKHKVYACEVTHQGLSSPVTKSFNRGEC

SEQ ID NO: 370 - protein, 258 aa, Artificial Sequence
  Spacer - YV24-2001 LC
QGQSGSCLHSAYNVCLDPGGGSSGGSISSGLLSGRSDNHGGGSEIVLTQSPGTLSLSPGERATLSCRASQSVGSSYLAWYQQKPGQAPRLLIYGAFSRATGIPDRFSGSGSGTDFTLTISRLEPEDFAVYYCQQYGSSPWTFGQGTKVEIKRTVAAPSVFIFPPSDEQLKSGTASVVCLLNNFYPREAKVQWKVDNALQSGNSQESVTEQDSKDSTYSLSSTLTLSKADYEKHKVYACEVTHQGLSSPVTKSFNRGEC

SEQ ID NO: 371 - protein, 252 aa, Artificial Sequence
  YV24-2001 LC
CLHSAYNVCLDPGGGSSGGSISSGLLSGRSDNHGGGSEIVLTQSPGTLSLSPGERATLSCRASQSVGSSYLAWYQQKPGQAPRLLIYGAFSRATGIPDRFSGSGSGTDFTLTISRLEPEDFAVYYCQQYGSSPWTFGQGTKVEIKRTVAAPSVFIFPPSDEQLKSGTASVVCLLNNFYPREAKVQWKVDNALQSGNSQESVTEQDSKDSTYSLSSTLTLSKADYEKHKVYACEVTHQGLSSPVTKSFNRGEC

SEQ ID NO: 372 - protein, 258 aa, Artificial Sequence
  Spacer - YV27-2001 LC
QGQSGSQPCAQMYGYSMCGGGSSGGSISSGLLSGRSDNHGGGSEIVLTQSPGTLSLSPGERATLSCRASQSVGSSYLAWYQQKPGQAPRLLIYGAFSRATGIPDRFSGSGSGTDFTLTISRLEPEDFAVYYCQQYGSSPWTFGQGTKVEIKRTVAAPSVFIFPPSDEQLKSGTASVVCLLNNFYPREAKVQWKVDNALQSGNSQESVTEQDSKDSTYSLSSTLTLSKADYEKHKVYACEVTHQGLSSPVTKSFNRGEC

SEQ ID NO: 373 - protein, 252 aa, Artificial Sequence
  YV27-2001 LC
QPCAQMYGYSMCGGGSSGGSISSGLLSGRSDNHGGGSEIVLTQSPGTLSLSPGERATLSCRASQSVGSSYLAWYQQKPGQAPRLLIYGAFSRATGIPDRFSGSGSGTDFTLTISRLEPEDFAVYYCQQYGSSPWTFGQGTKVEIKRTVAAPSVFIFPPSDEQLKSGTASVVCLLNNFYPREAKVQWKVDNALQSGNSQESVTEQDSKDSTYSLSSTLTLSKADYEKHKVYACEVTHQGLSSPVTKSFNRGEC

SEQ ID NO: 374 - protein, 259 aa, Artificial Sequence
  Spacer - YV29-2001 LC
QGQSGSCAQMYGYSMCAHTGGGSSGGSISSGLLSGRSDNHGGGSEIVLTQSPGTLSLSPGERATLSCRASQSVGSSYLAWYQQKPGQAPRLLIYGAFSRATGIPDRFSGSGSGTDFTLTISRLEPEDFAVYYCQQYGSSPWTFGQGTKVEIKRTVAAPSVFIFPPSDEQLKSGTASVVCLLNNFYPREAKVQWKVDNALQSGNSQESVTEQDSKDSTYSLSSTLTLSKADYEKHKVYACEVTHQGLSSPVTKSFNRGEC

SEQ ID NO: 375 - protein, 253 aa, Artificial Sequence
  YV29-2001 LC
CAQMYGYSMCAHTGGGSSGGSISSGLLSGRSDNHGGGSEIVLTQSPGTLSLSPGERATLSCRASQSVGSSYLAWYQQKPGQAPRLLIYGAFSRATGIPDRFSGSGSGTDFTLTISRLEPEDFAVYYCQQYGSSPWTFGQGTKVEIKRTVAAPSVFIFPPSDEQLKSGTASVVCLLNNFYPREAKVQWKVDNALQSGNSQESVTEQDSKDSTYSLSSTLTLSKADYEKHKVYACEVTHQGLSSPVTKSFNRGEC

SEQ ID NO: 376 - protein, 257 aa, Artificial Sequence
  Spacer - YV32-2001 LC
QGQSGSCPNHPLCHDWQGGGSSGGSISSGLLSGRSDNHGGGSEIVLTQSPGTLSLSPGERATLSCRASQSVGSSYLAWYQQKPGQAPRLLIYGAFSRATGIPDRFSGSGSGTDFTLTISRLEPEDFAVYYCQQYGSSPWTFGQGTKVEIKRTVAAPSVFIFPPSDEQLKSGTASVVCLLNNFYPREAKVQWKVDNALQSGNSQESVTEQDSKDSTYSLSSTLTLSKADYEKHKVYACEVTHQGLSSPVTKSFNRGEC

SEQ ID NO: 377 - protein, 251 aa, Artificial Sequence
  YV32-2001 LC
CPNHPLCHDWQGGGSSGGSISSGLLSGRSDNHGGGSEIVLTQSPGTLSLSPGERATLSCRASQSVGSSYLAWYQQKPGQAPRLLIYGAFSRATGIPDRFSGSGSGTDFTLTISRLEPEDFAVYYCQQYGSSPWTFGQGTKVEIKRTVAAPSVFIFPPSDEQLKSGTASVVCLLNNFYPREAKVQWKVDNALQSGNSQESVTEQDSKDSTYSLSSTLTLSKADYEKHKVYACEVTHQGLSSPVTKSFNRGEC

SEQ ID NO: 378 - protein, 257 aa, Artificial Sequence
  Spacer - YV33-2001 LC
QGQSGSCPNHPMCADWQGGGSSGGSISSGLLSGRSDNHGGGSEIVLTQSPGTLSLSPGERATLSCRASQSVGSSYLAWYQQKPGQAPRLLIYGAFSRATGIPDRFSGSGSGTDFTLTISRLEPEDFAVYYCQQYGSSPWTFGQGTKVEIKRTVAAPSVFIFPPSDEQLKSGTASVVCLLNNFYPREAKVQWKVDNALQSGNSQESVTEQDSKDSTYSLSSTLTLSKADYEKHKVYACEVTHQGLSSPVTKSFNRGEC

SEQ ID NO: 379 - protein, 251 aa, Artificial Sequence
  YV33-2001 LC
CPNHPMCADWQGGGSSGGSISSGLLSGRSDNHGGGSEIVLTQSPGTLSLSPGERATLSCRASQSVGSSYLAWYQQKPGQAPRLLIYGAFSRATGIPDRFSGSGSGTDFTLTISRLEPEDFAVYYCQQYGSSPWTFGQGTKVEIKRTVAAPSVFIFPPSDEQLKSGTASVVCLLNNFYPREAKVQWKVDNALQSGNSQESVTEQDSKDSTYSLSSTLTLSKADYEKHKVYACEVTHQGLSSPVTKSFNRGEC

SEQ ID NO: 380 - protein, 257 aa, Artificial Sequence
  Spacer - YV35-2001 LC
QGQSGSCPNHPMCHDAQGGGSSGGSISSGLLSGRSDNHGGGSEIVLTQSPGTLSLSPGERATLSCRASQSVGSSYLAWYQQKPGQAPRLLIYGAFSRATGIPDRFSGSGSGTDFTLTISRLEPEDFAVYYCQQYGSSPWTFGQGTKVEIKRTVAAPSVFIFPPSDEQLKSGTASVVCLLNNFYPREAKVQWKVDNALQSGNSQESVTEQDSKDSTYSLSSTLTLSKADYEKHKVYACEVTHQGLSSPVTKSFNRGEC

SEQ ID NO: 381 - protein, 251 aa, Artificial Sequence
  YV35-2001 LC
CPNHPMCHDAQGGGSSGGSISSGLLSGRSDNHGGGSEIVLTQSPGTLSLSPGERATLSCRASQSVGSSYLAWYQQKPGQAPRLLIYGAFSRATGIPDRFSGSGSGTDFTLTISRLEPEDFAVYYCQQYGSSPWTFGQGTKVEIKRTVAAPSVFIFPPSDEQLKSGTASVVCLLNNFYPREAKVQWKVDNALQSGNSQESVTEQDSKDSTYSLSSTLTLSKADYEKHKVYACEVTHQGLSSPVTKSFNRGEC

SEQ ID NO: 382 - protein, 259 aa, Artificial Sequence
  Spacer - YV39-2001 LC
QGQSGSCRTQLYGYNLCPYGGGSSGGSISSGLLSGRSDNHGGGSEIVLTQSPGTLSLSPGERATLSCRASQSVGSSYLAWYQQKPGQAPRLLIYGAFSRATGIPDRFSGSGSGTDFTLTISRLEPEDFAVYYCQQYGSSPWTFGQGTKVEIKRTVAAPSVFIFPPSDEQLKSGTASVVCLLNNFYPREAKVQWKVDNALQSGNSQESVTEQDSKDSTYSLSSTLTLSKADYEKHKVYACEVTHQGLSSPVTKSFNRGEC

SEQ ID NO: 383 - protein, 253 aa, Artificial Sequence
  YV39-2001 LC
CRTQLYGYNLCPYGGGSSGGSISSGLLSGRSDNHGGGSEIVLTQSPGTLSLSPGERATLSCRASQSVGSSYLAWYQQKPGQAPRLLIYGAFSRATGIPDRFSGSGSGTDFTLTISRLEPEDFAVYYCQQYGSSPWTFGQGTKVEIKRTVAAPSVFIFPPSDEQLKSGTASVVCLLNNFYPREAKVQWKVDNALQSGNSQESVTEQDSKDSTYSLSSTLTLSKADYEKHKVYACEVTHQGLSSPVTKSFNRGEC

SEQ ID NO: 384 - protein, 259 aa, Artificial Sequence
  Spacer - YV41-2001 LC
QGQSGSCRTQLYGYNLCPAGGGSSGGSISSGLLSGRSDNHGGGSEIVLTQSPGTLSLSPGERATLSCRASQSVGSSYLAWYQQKPGQAPRLLIYGAFSRATGIPDRFSGSGSGTDFTLTISRLEPEDFAVYYCQQYGSSPWTFGQGTKVEIKRTVAAPSVFIFPPSDEQLKSGTASVVCLLNNFYPREAKVQWKVDNALQSGNSQESVTEQDSKDSTYSLSSTLTLSKADYEKHKVYACEVTHQGLSSPVTKSFNRGEC

SEQ ID NO: 385 - protein, 253 aa, Artificial Sequence
  YV41-2001 LC
CRTQLYGYNLCPAGGGSSGGSISSGLLSGRSDNHGGGSEIVLTQSPGTLSLSPGERATLSCRASQSVGSSYLAWYQQKPGQAPRLLIYGAFSRATGIPDRFSGSGSGTDFTLTISRLEPEDFAVYYCQQYGSSPWTFGQGTKVEIKRTVAAPSVFIFPPSDEQLKSGTASVVCLLNNFYPREAKVQWKVDNALQSGNSQESVTEQDSKDSTYSLSSTLTLSKADYEKHKVYACEVTHQGLSSPVTKSFNRGEC

SEQ ID NO: 386 - protein, 261 aa, Artificial Sequence
  Spacer - YV51-2001 LC
QGQSGSFGAACPNHPICHDWQGGGSSGGSISSGLLSGRSDNHGGGSEIVLTQSPGTLSLSPGERATLSCRASQSVGSSYLAWYQQKPGQAPRLLIYGAFSRATGIPDRFSGSGSGTDFTLTISRLEPEDFAVYYCQQYGSSPWTFGQGTKVEIKRTVAAPSVFIFPPSDEQLKSGTASVVCLLNNFYPREAKVQWKVDNALQSGNSQESVTEQDSKDSTYSLSSTLTLSKADYEKHKVYACEVTHQGLSSPVTKSFNRGEC

SEQ ID NO: 387 - protein, 255 aa, Artificial Sequence
  YV51-2001 LC
FGAACPNHPICHDWQGGGSSGGSISSGLLSGRSDNHGGGSEIVLTQSPGTLSLSPGERATLSCRASQSVGSSYLAWYQQKPGQAPRLLIYGAFSRATGIPDRFSGSGSGTDFTLTISRLEPEDFAVYYCQQYGSSPWTFGQGTKVEIKRTVAAPSVFIFPPSDEQLKSGTASVVCLLNNFYPREAKVQWKVDNALQSGNSQESVTEQDSKDSTYSLSSTLTLSKADYEKHKVYACEVTHQGLSSPVTKSFNRGEC

SEQ ID NO: 388 - protein, 261 aa, Artificial Sequence
  Spacer - YV52-2001 LC
QGQSGSFGAACPNHPLCHDWQGGGSSGGSISSGLLSGRSDNHGGGSEIVLTQSPGTLSLSPGERATLSCRASQSVGSSYLAWYQQKPGQAPRLLIYGAFSRATGIPDRFSGSGSGTDFTLTISRLEPEDFAVYYCQQYGSSPWTFGQGTKVEIKRTVAAPSVFIFPPSDEQLKSGTASVVCLLNNFYPREAKVQWKVDNALQSGNSQESVTEQDSKDSTYSLSSTLTLSKADYEKHKVYACEVTHQGLSSPVTKSFNRGEC

SEQ ID NO: 389 - protein, 255 aa, Artificial Sequence
  YV52-2001 LC
FGAACPNHPLCHDWQGGGSSGGSISSGLLSGRSDNHGGGSEIVLTQSPGTLSLSPGERATLSCRASQSVGSSYLAWYQQKPGQAPRLLIYGAFSRATGIPDRFSGSGSGTDFTLTISRLEPEDFAVYYCQQYGSSPWTFGQGTKVEIKRTVAAPSVFIFPPSDEQLKSGTASVVCLLNNFYPREAKVQWKVDNALQSGNSQESVTEQDSKDSTYSLSSTLTLSKADYEKHKVYACEVTHQGLSSPVTKSFNRGEC

SEQ ID NO: 390 - protein, 261 aa, Artificial Sequence
  Spacer - YV53-2001 LC
QGQSGSFGAACPNHPMCHDAQGGGSSGGSISSGLLSGRSDNHGGGSEIVLTQSPGTLSLSPGERATLSCRASQSVGSSYLAWYQQKPGQAPRLLIYGAFSRATGIPDRFSGSGSGTDFTLTISRLEPEDFAVYYCQQYGSSPWTFGQGTKVEIKRTVAAPSVFIFPPSDEQLKSGTASVVCLLNNFYPREAKVQWKVDNALQSGNSQESVTEQDSKDSTYSLSSTLTLSKADYEKHKVYACEVTHQGLSSPVTKSFNRGEC

SEQ ID NO: 391 - protein, 255 aa, Artificial Sequence
  YV53-2001 LC
FGAACPNHPMCHDAQGGGSSGGSISSGLLSGRSDNHGGGSEIVLTQSPGTLSLSPGERATLSCRASQSVGSSYLAWYQQKPGQAPRLLIYGAFSRATGIPDRFSGSGSGTDFTLTISRLEPEDFAVYYCQQYGSSPWTFGQGTKVEIKRTVAAPSVFIFPPSDEQLKSGTASVVCLLNNFYPREAKVQWKVDNALQSGNSQESVTEQDSKDSTYSLSSTLTLSKADYEKHKVYACEVTHQGLSSPVTKSFNRGEC

SEQ ID NO: 392 - protein, 258 aa, Artificial Sequence
  Spacer - YV54-2001 LC
QGQSGSCLHSAYNACLDPGGGSSGGSISSGLLSGRSDNHGGGSEIVLTQSPGTLSLSPGERATLSCRASQSVGSSYLAWYQQKPGQAPRLLIYGAFSRATGIPDRFSGSGSGTDFTLTISRLEPEDFAVYYCQQYGSSPWTFGQGTKVEIKRTVAAPSVFIFPPSDEQLKSGTASVVCLLNNFYPREAKVQWKVDNALQSGNSQESVTEQDSKDSTYSLSSTLTLSKADYEKHKVYACEVTHQGLSSPVTKSFNRGEC

SEQ ID NO: 393 - protein, 252 aa, Artificial Sequence
  YV54-2001 LC
CLHSAYNACLDPGGGSSGGSISSGLLSGRSDNHGGGSEIVLTQSPGTLSLSPGERATLSCRASQSVGSSYLAWYQQKPGQAPRLLIYGAFSRATGIPDRFSGSGSGTDFTLTISRLEPEDFAVYYCQQYGSSPWTFGQGTKVEIKRTVAAPSVFIFPPSDEQLKSGTASVVCLLNNFYPREAKVQWKVDNALQSGNSQESVTEQDSKDSTYSLSSTLTLSKADYEKHKVYACEVTHQGLSSPVTKSFNRGEC

SEQ ID NO: 394 - protein, 258 aa, Artificial Sequence
  Spacer - YV55-2001 LC
QGQSGSCAHSAYNVCLDPGGGSSGGSISSGLLSGRSDNHGGGSEIVLTQSPGTLSLSPGERATLSCRASQSVGSSYLAWYQQKPGQAPRLLIYGAFSRATGIPDRFSGSGSGTDFTLTISRLEPEDFAVYYCQQYGSSPWTFGQGTKVEIKRTVAAPSVFIFPPSDEQLKSGTASVVCLLNNFYPREAKVQWKVDNALQSGNSQESVTEQDSKDSTYSLSSTLTLSKADYEKHKVYACEVTHQGLSSPVTKSFNRGEC

SEQ ID NO: 395 - protein, 252 aa, Artificial Sequence
  YV55-2001 LC
CAHSAYNVCLDPGGGSSGGSISSGLLSGRSDNHGGGSEIVLTQSPGTLSLSPGERATLSCRASQSVGSSYLAWYQQKPGQAPRLLIYGAFSRATGIPDRFSGSGSGTDFTLTISRLEPEDFAVYYCQQYGSSPWTFGQGTKVEIKRTVAAPSVFIFPPSDEQLKSGTASVVCLLNNFYPREAKVQWKVDNALQSGNSQESVTEQDSKDSTYSLSSTLTLSKADYEKHKVYACEVTHQGLSSPVTKSFNRGEC

SEQ ID NO: 396 - protein, 258 aa, Artificial Sequence
  Spacer - YV56-2001 LC
QGQSGSCLHSAYNVCADPGGGSSGGSISSGLLSGRSDNHGGGSEIVLTQSPGTLSLSPGERATLSCRASQSVGSSYLAWYQQKPGQAPRLLIYGAFSRATGIPDRFSGSGSGTDFTLTISRLEPEDFAVYYCQQYGSSPWTFGQGTKVEIKRTVAAPSVFIFPPSDEQLKSGTASVVCLLNNFYPREAKVQWKVDNALQSGNSQESVTEQDSKDSTYSLSSTLTLSKADYEKHKVYACEVTHQGLSSPVTKSFNRGEC

SEQ ID NO: 397 - protein, 252 aa, Artificial Sequence
  YV56-2001 LC
CLHSAYNVCADPGGGSSGGSISSGLLSGRSDNHGGGSEIVLTQSPGTLSLSPGERATLSCRASQSVGSSYLAWYQQKPGQAPRLLIYGAFSRATGIPDRFSGSGSGTDFTLTISRLEPEDFAVYYCQQYGSSPWTFGQGTKVEIKRTVAAPSVFIFPPSDEQLKSGTASVVCLLNNFYPREAKVQWKVDNALQSGNSQESVTEQDSKDSTYSLSSTLTLSKADYEKHKVYACEVTHQGLSSPVTKSFNRGEC

SEQ ID NO: 398 - protein, 258 aa, Artificial Sequence
  Spacer - YV57-2001 LC
QGQSGSCLHSAYNVCLAPGGGSSGGSISSGLLSGRSDNHGGGSEIVLTQSPGTLSLSPGERATLSCRASQSVGSSYLAWYQQKPGQAPRLLIYGAFSRATGIPDRFSGSGSGTDFTLTISRLEPEDFAVYYCQQYGSSPWTFGQGTKVEIKRTVAAPSVFIFPPSDEQLKSGTASVVCLLNNFYPREAKVQWKVDNALQSGNSQESVTEQDSKDSTYSLSSTLTLSKADYEKHKVYACEVTHQGLSSPVTKSFNRGEC

SEQ ID NO: 399 - protein, 252 aa, Artificial Sequence
  YV57-2001 LC
CLHSAYNVCLAPGGGSSGGSISSGLLSGRSDNHGGGSEIVLTQSPGTLSLSPGERATLSCRASQSVGSSYLAWYQQKPGQAPRLLIYGAFSRATGIPDRFSGSGSGTDFTLTISRLEPEDFAVYYCQQYGSSPWTFGQGTKVEIKRTVAAPSVFIFPPSDEQLKSGTASVVCLLNNFYPREAKVQWKVDNALQSGNSQESVTEQDSKDSTYSLSSTLTLSKADYEKHKVYACEVTHQGLSSPVTKSFNRGEC

SEQ ID NO: 400 - protein, 258 aa, Artificial Sequence
  Spacer - YV58-2001 LC
QGQSGSCLHSAYNVCLDAGGGSSGGSISSGLLSGRSDNHGGGSEIVLTQSPGTLSLSPGERATLSCRASQSVGSSYLAWYQQKPGQAPRLLIYGAFSRATGIPDRFSGSGSGTDFTLTISRLEPEDFAVYYCQQYGSSPWTFGQGTKVEIKRTVAAPSVFIFPPSDEQLKSGTASVVCLLNNFYPREAKVQWKVDNALQSGNSQESVTEQDSKDSTYSLSSTLTLSKADYEKHKVYACEVTHQGLSSPVTKSFNRGEC

SEQ ID NO: 401 - protein, 252 aa, Artificial Sequence
  YV58-2001 LC
CLHSAYNVCLDAGGGSSGGSISSGLLSGRSDNHGGGSEIVLTQSPGTLSLSPGERATLSCRASQSVGSSYLAWYQQKPGQAPRLLIYGAFSRATGIPDRFSGSGSGTDFTLTISRLEPEDFAVYYCQQYGSSPWTFGQGTKVEIKRTVAAPSVFIFPPSDEQLKSGTASVVCLLNNFYPREAKVQWKVDNALQSGNSQESVTEQDSKDSTYSLSSTLTLSKADYEKHKVYACEVTHQGLSSPVTKSFNRGEC

SEQ ID NO: 402 - protein, 261 aa, Artificial Sequence
  Spacer - YV61-2001 LC
QGQSGSYISDCPYHPMCHDYQGGGSSGGSISSGLLSGRSDNHGGGSEIVLTQSPGTLSLSPGERATLSCRASQSVGSSYLAWYQQKPGQAPRLLIYGAFSRATGIPDRFSGSGSGTDFTLTISRLEPEDFAVYYCQQYGSSPWTFGQGTKVEIKRTVAAPSVFIFPPSDEQLKSGTASVVCLLNNFYPREAKVQWKVDNALQSGNSQESVTEQDSKDSTYSLSSTLTLSKADYEKHKVYACEVTHQGLSSPVTKSFNRGEC

SEQ ID NO: 403 - protein, 255 aa, Artificial Sequence
  YV61-2001 LC
YISDCPYHPMCHDYQGGGSSGGSISSGLLSGRSDNHGGGSEIVLTQSPGTLSLSPGERATLSCRASQSVGSSYLAWYQQKPGQAPRLLIYGAFSRATGIPDRFSGSGSGTDFTLTISRLEPEDFAVYYCQQYGSSPWTFGQGTKVEIKRTVAAPSVFIFPPSDEQLKSGTASVVCLLNNFYPREAKVQWKVDNALQSGNSQESVTEQDSKDSTYSLSSTLTLSKADYEKHKVYACEVTHQGLSSPVTKSFNRGEC

SEQ ID NO: 404 - protein, 261 aa, Artificial Sequence
  Spacer - YV62-2001 LC
QGQSGSFRNTCPYHPMCHDYRGGGSSGGSISSGLLSGRSDNHGGGSEIVLTQSPGTLSLSPGERATLSCRASQSVGSSYLAWYQQKPGQAPRLLIYGAFSRATGIPDRFSGSGSGTDFTLTISRLEPEDFAVYYCQQYGSSPWTFGQGTKVEIKRTVAAPSVFIFPPSDEQLKSGTASVVCLLNNFYPREAKVQWKVDNALQSGNSQESVTEQDSKDSTYSLSSTLTLSKADYEKHKVYACEVTHQGLSSPVTKSFNRGEC

SEQ ID NO: 405 - protein, 255 aa, Artificial Sequence
  YV62-2001 LC
FRNTCPYHPMCHDYRGGGSSGGSISSGLLSGRSDNHGGGSEIVLTQSPGTLSLSPGERATLSCRASQSVGSSYLAWYQQKPGQAPRLLIYGAFSRATGIPDRFSGSGSGTDFTLTISRLEPEDFAVYYCQQYGSSPWTFGQGTKVEIKRTVAAPSVFIFPPSDEQLKSGTASVVCLLNNFYPREAKVQWKVDNALQSGNSQESVTEQDSKDSTYSLSSTLTLSKADYEKHKVYACEVTHQGLSSPVTKSFNRGEC

SEQ ID NO: 406 - protein, 261 aa, Artificial Sequence
  Spacer - YV63-2001 LC
QGQSGSRECHMWMFGVNLCPYGGGSSGGSISSGLLSGRSDNHGGGSEIVLTQSPGTLSLSPGERATLSCRASQSVGSSYLAWYQQKPGQAPRLLIYGAFSRATGIPDRFSGSGSGTDFTLTISRLEPEDFAVYYCQQYGSSPWTFGQGTKVEIKRTVAAPSVFIFPPSDEQLKSGTASVVCLLNNFYPREAKVQWKVDNALQSGNSQESVTEQDSKDSTYSLSSTLTLSKADYEKHKVYACEVTHQGLSSPVTKSFNRGEC

SEQ ID NO: 407 - protein, 255 aa, Artificial Sequence
  YV63-2001 LC
RECHMWMFGVNLCPYGGGSSGGSISSGLLSGRSDNHGGGSEIVLTQSPGTLSLSPGERATLSCRASQSVGSSYLAWYQQKPGQAPRLLIYGAFSRATGIPDRFSGSGSGTDFTLTISRLEPEDFAVYYCQQYGSSPWTFGQGTKVEIKRTVAAPSVFIFPPSDEQLKSGTASVVCLLNNFYPREAKVQWKVDNALQSGNSQESVTEQDSKDSTYSLSSTLTLSKADYEKHKVYACEVTHQGLSSPVTKSFNRGEC

SEQ ID NO: 408 - protein, 261 aa, Artificial Sequence
  Spacer - YV64-2001 LC
QGQSGSAVCHMYMYGYNLCPFGGGSSGGSISSGLLSGRSDNHGGGSEIVLTQSPGTLSLSPGERATLSCRASQSVGSSYLAWYQQKPGQAPRLLIYGAFSRATGIPDRFSGSGSGTDFTLTISRLEPEDFAVYYCQQYGSSPWTFGQGTKVEIKRTVAAPSVFIFPPSDEQLKSGTASVVCLLNNFYPREAKVQWKVDNALQSGNSQESVTEQDSKDSTYSLSSTLTLSKADYEKHKVYACEVTHQGLSSPVTKSFNRGEC

SEQ ID NO: 409 - protein, 255 aa, Artificial Sequence
  YV64-2001 LC
AVCHMYMYGYNLCPFGGGSSGGSISSGLLSGRSDNHGGGSEIVLTQSPGTLSLSPGERATLSCRASQSVGSSYLAWYQQKPGQAPRLLIYGAFSRATGIPDRFSGSGSGTDFTLTISRLEPEDFAVYYCQQYGSSPWTFGQGTKVEIKRTVAAPSVFIFPPSDEQLKSGTASVVCLLNNFYPREAKVQWKVDNALQSGNSQESVTEQDSKDSTYSLSSTLTLSKADYEKHKVYACEVTHQGLSSPVTKSFNRGEC

SEQ ID NO: 410 - protein, 262 aa, Artificial Sequence
  Spacer - YV65-2001 LC
QGQSGQGRSCPQMYGYSMCPHTGGGSSGGSISSGLLSGRSDNHGGGSEIVLTQSPGTLSLSPGERATLSCRASQSVGSSYLAWYQQKPGQAPRLLIYGAFSRATGIPDRFSGSGSGTDFTLTISRLEPEDFAVYYCQQYGSSPWTFGQGTKVEIKRTVAAPSVFIFPPSDEQLKSGTASVVCLLNNFYPREAKVQWKVDNALQSGNSQESVTEQDSKDSTYSLSSTLTLSKADYEKHKVYACEVTHQGLSSPVTKSFNRGEC

SEQ ID NO: 411 - protein, 255 aa, Artificial Sequence
  YV65-2001 LC
RSCPQMYGYSMCPHTGGGSSGGSISSGLLSGRSDNHGGGSEIVLTQSPGTLSLSPGERATLSCRASQSVGSSYLAWYQQKPGQAPRLLIYGAFSRATGIPDRFSGSGSGTDFTLTISRLEPEDFAVYYCQQYGSSPWTFGQGTKVEIKRTVAAPSVFIFPPSDEQLKSGTASVVCLLNNFYPREAKVQWKVDNALQSGNSQESVTEQDSKDSTYSLSSTLTLSKADYEKHKVYACEVTHQGLSSPVTKSFNRGEC

SEQ ID NO: 412 - protein, 262 aa, Artificial Sequence
  Spacer - YV66-2001 LC
QGQSGQGQPCAQMFGYSMCPHTGGGSSGGSISSGLLSGRSDNHGGGSEIVLTQSPGTLSLSPGERATLSCRASQSVGSSYLAWYQQKPGQAPRLLIYGAFSRATGIPDRFSGSGSGTDFTLTISRLEPEDFAVYYCQQYGSSPWTFGQGTKVEIKRTVAAPSVFIFPPSDEQLKSGTASVVCLLNNFYPREAKVQWKVDNALQSGNSQESVTEQDSKDSTYSLSSTLTLSKADYEKHKVYACEVTHQGLSSPVTKSFNRGEC

SEQ ID NO: 413 - protein, 255 aa, Artificial Sequence
  YV66-2001 LC
QPCAQMFGYSMCPHTGGGSSGGSISSGLLSGRSDNHGGGSEIVLTQSPGTLSLSPGERATLSCRASQSVGSSYLAWYQQKPGQAPRLLIYGAFSRATGIPDRFSGSGSGTDFTLTISRLEPEDFAVYYCQQYGSSPWTFGQGTKVEIKRTVAAPSVFIFPPSDEQLKSGTASVVCLLNNFYPREAKVQWKVDNALQSGNSQESVTEQDSKDSTYSLSSTLTLSKADYEKHKVYACEVTHQGLSSPVTKSFNRGEC

SEQ ID NO: 414 - protein, 262 aa, Artificial Sequence
  Spacer - YV04-2006 LC
QGQSGSLHCRTQLYGYNLCPYGGGSSGGSISSGLLSGRSDDHGGGSEIVLTQSPGTLSLSPGERATLSCRASQSVGSSYLAWYQQKPGQAPRLLIYGAFSRATGIPDRFSGSGSGTDFTLTISRLEPEDFAVYYCQQYGSSPWTFGQGTKVEIKRTVAAPSVFIFPPSDEQLKSGTASVVCLLNNFYPREAKVQWKVDNALQSGNSQESVTEQDSKDSTYSLSSTLTLSKADYEKHKVYACEVTHQGLSSPVTKSFNRGECC

SEQ ID NO: 415 - protein, 255 aa, Artificial Sequence
  YV04-2006 LC
LHCRTQLYGYNLCPYGGGSSGGSISSGLLSGRSDDHGGGSEIVLTQSPGTLSLSPGERATLSCRASQSVGSSYLAWYQQKPGQAPRLLIYGAFSRATGIPDRFSGSGSGTDFTLTISRLEPEDFAVYYCQQYGSSPWTFGQGTKVEIKRTVAAPSVFIFPPSDEQLKSGTASVVCLLNNFYPREAKVQWKVDNALQSGNSQESVTEQDSKDSTYSLSSTLTLSKADYEKHKVYACEVTHQGLSSPVTKSFNRGEC

SEQ ID NO: 416 - protein, 258 aa, Artificial Sequence
  Spacer - YV23-2006 LC
QGQSGSCLHSLYNVCLDPGGGSSGGSISSGLLSGRSDDHGGGSEIVLTQSPGTLSLSPGERATLSCRASQSVGSSYLAWYQQKPGQAPRLLIYGAFSRATGIPDRFSGSGSGTDFTLTISRLEPEDFAVYYCQQYGSSPWTFGQGTKVEIKRTVAAPSVFIFPPSDEQLKSGTASVVCLLNNFYPREAKVQWKVDNALQSGNSQESVTEQDSKDSTYSLSSTLTLSKADYEKHKVYACEVTHQGLSSPVTKSFNRGEC

SEQ ID NO: 417 - protein, 252 aa, Artificial Sequence
  YV23-2006 LC
CLHSLYNVCLDPGGGSSGGSISSGLLSGRSDDHGGGSEIVLTQSPGTLSLSPGERATLSCRASQSVGSSYLAWYQQKPGQAPRLLIYGAFSRATGIPDRFSGSGSGTDFTLTISRLEPEDFAVYYCQQYGSSPWTFGQGTKVEIKRTVAAPSVFIFPPSDEQLKSGTASVVCLLNNFYPREAKVQWKVDNALQSGNSQESVTEQDSKDSTYSLSSTLTLSKADYEKHKVYACEVTHQGLSSPVTKSFNRGEC

SEQ ID NO: 418 - protein, 259 aa, Artificial Sequence
  Spacer - YV39-2006 LC
QGQSGSCRTQLYGYNLCPYGGGSSGGSISSGLLSGRSDDHGGGSEIVLTQSPGTLSLSPGERATLSCRASQSVGSSYLAWYQQKPGQAPRLLIYGAFSRATGIPDRFSGSGSGTDFTLTISRLEPEDFAVYYCQQYGSSPWTFGQGTKVEIKRTVAAPSVFIFPPSDEQLKSGTASVVCLLNNFYPREAKVQWKVDNALQSGNSQESVTEQDSKDSTYSLSSTLTLSKADYEKHKVYACEVTHQGLSSPVTKSFNRGEC

SEQ ID NO: 419 - protein, 253 aa, Artificial Sequence
  YV39-2006 LC
CRTQLYGYNLCPYGGGSSGGSISSGLLSGRSDDHGGGSEIVLTQSPGTLSLSPGERATLSCRASQSVGSSYLAWYQQKPGQAPRLLIYGAFSRATGIPDRFSGSGSGTDFTLTISRLEPEDFAVYYCQQYGSSPWTFGQGTKVEIKRTVAAPSVFIFPPSDEQLKSGTASVVCLLNNFYPREAKVQWKVDNALQSGNSQESVTEQDSKDSTYSLSSTLTLSKADYEKHKVYACEVTHQGLSSPVTKSFNRGEC

SEQ ID NO: 420 - protein, 261 aa, Artificial Sequence
  Spacer - YV04-2007 LC
QGQSGSLHCRTQLYGYNLCPYGGGSSGGSISSGLLSGRSDIHGGGSEIVLTQSPGTLSLSPGERATLSCRASQSVGSSYLAWYQQKPGQAPRLLIYGAFSRATGIPDRFSGSGSGTDFTLTISRLEPEDFAVYYCQQYGSSPWTFGQGTKVEIKRTVAAPSVFIFPPSDEQLKSGTASVVCLLNNFYPREAKVQWKVDNALQSGNSQESVTEQDSKDSTYSLSSTLTLSKADYEKHKVYACEVTHQGLSSPVTKSFNRGEC

SEQ ID NO: 421 - protein, 255 aa, Artificial Sequence
  YV04-2007 LC
LHCRTQLYGYNLCPYGGGSSGGSISSGLLSGRSDIHGGGSEIVLTQSPGTLSLSPGERATLSCRASQSVGSSYLAWYQQKPGQAPRLLIYGAFSRATGIPDRFSGSGSGTDFTLTISRLEPEDFAVYYCQQYGSSPWTFGQGTKVEIKRTVAAPSVFIFPPSDEQLKSGTASVVCLLNNFYPREAKVQWKVDNALQSGNSQESVTEQDSKDSTYSLSSTLTLSKADYEKHKVYACEVTHQGLSSPVTKSFNRGEC

SEQ ID NO: 422 - protein, 258 aa, Artificial Sequence
  Spacer - YV23-2007 LC
QGQSGSCLHSLYNVCLDPGGGSSGGSISSGLLSGRSDIHGGGSEIVLTQSPGTLSLSPGERATLSCRASQSVGSSYLAWYQQKPGQAPRLLIYGAFSRATGIPDRFSGSGSGTDFTLTISRLEPEDFAVYYCQQYGSSPWTFGQGTKVEIKRTVAAPSVFIFPPSDEQLKSGTASVVCLLNNFYPREAKVQWKVDNALQSGNSQESVTEQDSKDSTYSLSSTLTLSKADYEKHKVYACEVTHQGLSSPVTKSFNRGEC

SEQ ID NO: 423 - protein, 252 aa, Artificial Sequence
  YV23-2007 LC
CLHSLYNVCLDPGGGSSGGSISSGLLSGRSDIHGGGSEIVLTQSPGTLSLSPGERATLSCRASQSVGSSYLAWYQQKPGQAPRLLIYGAFSRATGIPDRFSGSGSGTDFTLTISRLEPEDFAVYYCQQYGSSPWTFGQGTKVEIKRTVAAPSVFIFPPSDEQLKSGTASVVCLLNNFYPREAKVQWKVDNALQSGNSQESVTEQDSKDSTYSLSSTLTLSKADYEKHKVYACEVTHQGLSSPVTKSFNRGEC

SEQ ID NO: 424 - protein, 259 aa, Artificial Sequence
  Spacer - YV39-2007 LC
QGQSGSCRTQLYGYNLCPYGGGSSGGSISSGLLSGRSDIHGGGSEIVLTQSPGTLSLSPGERATLSCRASQSVGSSYLAWYQQKPGQAPRLLIYGAFSRATGIPDRFSGSGSGTDFTLTISRLEPEDFAVYYCQQYGSSPWTFGQGTKVEIKRTVAAPSVFIFPPSDEQLKSGTASVVCLLNNFYPREAKVQWKVDNALQSGNSQESVTEQDSKDSTYSLSSTLTLSKADYEKHKVYACEVTHQGLSSPVTKSFNRGEC

SEQ ID NO: 425 - protein, 253 aa, Artificial Sequence
  YV39-2007 LC
CRTQLYGYNLCPYGGGSSGGSISSGLLSGRSDIHGGGSEIVLTQSPGTLSLSPGERATLSCRASQSVGSSYLAWYQQKPGQAPRLLIYGAFSRATGIPDRFSGSGSGTDFTLTISRLEPEDFAVYYCQQYGSSPWTFGQGTKVEIKRTVAAPSVFIFPPSDEQLKSGTASVVCLLNNFYPREAKVQWKVDNALQSGNSQESVTEQDSKDSTYSLSSTLTLSKADYEKHKVYACEVTHQGLSSPVTKSFNRGEC

SEQ ID NO: 426 - protein, 261 aa, Artificial Sequence
  Spacer - YV04-2008 LC
QGQSGSLHCRTQLYGYNLCPYGGGSSGGSISSGLLSGRSDQHGGGSEIVLTQSPGTLSLSPGERATLSCRASQSVGSSYLAWYQQKPGQAPRLLIYGAFSRATGIPDRFSGSGSGTDFTLTISRLEPEDFAVYYCQQYGSSPWTFGQGTKVEIKRTVAAPSVFIFPPSDEQLKSGTASVVCLLNNFYPREAKVQWKVDNALQSGNSQESVTEQDSKDSTYSLSSTLTLSKADYEKHKVYACEVTHQGLSSPVTKSFNRGEC

SEQ ID NO: 427 - protein, 255 aa, Artificial Sequence
  YV04-2008 LC
LHCRTQLYGYNLCPYGGGSSGGSISSGLLSGRSDQHGGGSEIVLTQSPGTLSLSPGERATLSCRASQSVGSSYLAWYQQKPGQAPRLLIYGAFSRATGIPDRFSGSGSGTDFTLTISRLEPEDFAVYYCQQYGSSPWTFGQGTKVEIKRTVAAPSVFIFPPSDEQLKSGTASVVCLLNNFYPREAKVQWKVDNALQSGNSQESVTEQDSKDSTYSLSSTLTLSKADYEKHKVYACEVTHQGLSSPVTKSFNRGEC

SEQ ID NO: 428 - protein, 258 aa, Artificial Sequence
  Spacer - YV23-2008 LC
QGQSGSCLHSLYNVCLDPGGGSSGGSISSGLLSGRSDQHGGGSEIVLTQSPGTLSLSPGERATLSCRASQSVGSSYLAWYQQKPGQAPRLLIYGAFSRATGIPDRFSGSGSGTDFTLTISRLEPEDFAVYYCQQYGSSPWTFGQGTKVEIKRTVAAPSVFIFPPSDEQLKSGTASVVCLLNNFYPREAKVQWKVDNALQSGNSQESVTEQDSKDSTYSLSSTLTLSKADYEKHKVYACEVTHQGLSSPVTKSFNRGEC

SEQ ID NO: 429 - protein, 252 aa, Artificial Sequence
  YV23-2008 LC
CLHSLYNVCLDPGGGSSGGSISSGLLSGRSDQHGGGSEIVLTQSPGTLSLSPGERATLSCRASQSVGSSYLAWYQQKPGQAPRLLIYGAFSRATGIPDRFSGSGSGTDFTLTISRLEPEDFAVYYCQQYGSSPWTFGQGTKVEIKRTVAAPSVFIFPPSDEQLKSGTASVVCLLNNFYPREAKVQWKVDNALQSGNSQESVTEQDSKDSTYSLSSTLTLSKADYEKHKVYACEVTHQGLSSPVTKSFNRGEC

SEQ ID NO: 430 - protein, 259 aa, Artificial Sequence
  Spacer - YV39-2008 LC
QGQSGSCRTQLYGYNLCPYGGGSSGGSISSGLLSGRSDQHGGGSEIVLTQSPGTLSLSPGERATLSCRASQSVGSSYLAWYQQKPGQAPRLLIYGAFSRATGIPDRFSGSGSGTDFTLTISRLEPEDFAVYYCQQYGSSPWTFGQGTKVEIKRTVAAPSVFIFPPSDEQLKSGTASVVCLLNNFYPREAKVQWKVDNALQSGNSQESVTEQDSKDSTYSLSSTLTLSKADYEKHKVYACEVTHQGLSSPVTKSFNRGEC

SEQ ID NO: 431 - protein, 253 aa, Artificial Sequence
  YV39-2008 LC
CRTQLYGYNLCPYGGGSSGGSISSGLLSGRSDQHGGGSEIVLTQSPGTLSLSPGERATLSCRASQSVGSSYLAWYQQKPGQAPRLLIYGAFSRATGIPDRFSGSGSGTDFTLTISRLEPEDFAVYYCQQYGSSPWTFGQGTKVEIKRTVAAPSVFIFPPSDEQLKSGTASVVCLLNNFYPREAKVQWKVDNALQSGNSQESVTEQDSKDSTYSLSSTLTLSKADYEKHKVYACEVTHQGLSSPVTKSFNRGEC

SEQ ID NO: 432 - protein, 259 aa, Artificial Sequence
  Spacer - YV04-2009 LC
QGQSGSLHCRTQLYGYNLCPYGSSGGSISSGLLSGRSDTHGGGSEIVLTQSPGTLSLSPGERATLSCRASQSVGSSYLAWYQQKPGQAPRLLIYGAFSRATGIPDRFSGSGSGTDFTLTISRLEPEDFAVYYCQQYGSSPWTFGQGTKVEIKRTVAAPSVFIFPPSDEQLKSGTASVVCLLNNFYPREAKVQWKVDNALQSGNSQESVTEQDSKDSTYSLSSTLTLSKADYEKHKVYACEVTHQGLSSPVTKSFNRGEC

SEQ ID NO: 433 - protein, 253 aa, Artificial Sequence
  YV04-2009 LC
LHCRTQLYGYNLCPYGSSGGSISSGLLSGRSDTHGGGSEIVLTQSPGTLSLSPGERATLSCRASQSVGSSYLAWYQQKPGQAPRLLIYGAFSRATGIPDRFSGSGSGTDFTLTISRLEPEDFAVYYCQQYGSSPWTFGQGTKVEIKRTVAAPSVFIFPPSDEQLKSGTASVVCLLNNFYPREAKVQWKVDNALQSGNSQESVTEQDSKDSTYSLSSTLTLSKADYEKHKVYACEVTHQGLSSPVTKSFNRGEC

SEQ ID NO: 434 - protein, 256 aa, Artificial Sequence
  Spacer - YV23-2009 LC
QGQSGSCLHSLYNVCLDPGSSGGSISSGLLSGRSDTHGGGSEIVLTQSPGTLSLSPGERATLSCRASQSVGSSYLAWYQQKPGQAPRLLIYGAFSRATGIPDRFSGSGSGTDFTLTISRLEPEDFAVYYCQQYGSSPWTFGQGTKVEIKRTVAAPSVFIFPPSDEQLKSGTASVVCLLNNFYPREAKVQWKVDNALQSGNSQESVTEQDSKDSTYSLSSTLTLSKADYEKHKVYACEVTHQGLSSPVTKSFNRGEC

SEQ ID NO: 435 - protein, 250 aa, Artificial Sequence
  YV23-2009 LC
CLHSLYNVCLDPGSSGGSISSGLLSGRSDTHGGGSEIVLTQSPGTLSLSPGERATLSCRASQSVGSSYLAWYQQKPGQAPRLLIYGAFSRATGIPDRFSGSGSGTDFTLTISRLEPEDFAVYYCQQYGSSPWTFGQGTKVEIKRTVAAPSVFIFPPSDEQLKSGTASVVCLLNNFYPREAKVQWKVDNALQSGNSQESVTEQDSKDSTYSLSSTLTLSKADYEKHKVYACEVTHQGLSSPVTKSFNRGEC

SEQ ID NO: 436 - protein, 259 aa, Artificial Sequence
  Spacer - YV39-2009 LC
QGQSGSCRTQLYGYNLCPYGGGSSGGSISSGLLSGRSDTHGGGSEIVLTQSPGTLSLSPGERATLSCRASQSVGSSYLAWYQQKPGQAPRLLIYGAFSRATGIPDRFSGSGSGTDFTLTISRLEPEDFAVYYCQQYGSSPWTFGQGTKVEIKRTVAAPSVFIFPPSDEQLKSGTASVVCLLNNFYPREAKVQWKVDNALQSGNSQESVTEQDSKDSTYSLSSTLTLSKADYEKHKVYACEVTHQGLSSPVTKSFNRGEC

SEQ ID NO: 437 - protein, 253 aa, Artificial Sequence
  YV39-2009 LC
CRTQLYGYNLCPYGGGSSGGSISSGLLSGRSDTHGGGSEIVLTQSPGTLSLSPGERATLSCRASQSVGSSYLAWYQQKPGQAPRLLIYGAFSRATGIPDRFSGSGSGTDFTLTISRLEPEDFAVYYCQQYGSSPWTFGQGTKVEIKRTVAAPSVFIFPPSDEQLKSGTASVVCLLNNFYPREAKVQWKVDNALQSGNSQESVTEQDSKDSTYSLSSTLTLSKADYEKHKVYACEVTHQGLSSPVTKSFNRGEC

SEQ ID NO: 438 - protein, 263 aa, Artificial Sequence
  Spacer - YV01-2011 LC
QGQSGQGDFSCLHSMYNVCLDPGGGSSGGSISSGLLSGRSDNPGGGSEIVLTQSPGTLSLSPGERATLSCRASQSVGSSYLAWYQQKPGQAPRLLIYGAFSRATGIPDRFSGSGSGTDFTLTISRLEPEDFAVYYCQQYGSSPWTFGQGTKVEIKRTVAAPSVFIFPPSDEQLKSGTASVVCLLNNFYPREAKVQWKVDNALQSGNSQESVTEQDSKDSTYSLSSTLTLSKADYEKHKVYACEVTHQGLSSPVTKSFNRGECC

SEQ ID NO: 439 - protein, 255 aa, Artificial Sequence
  YV01-2011 LC
DFSCLHSMYNVCLDPGGGSSGGSISSGLLSGRSDNPGGGSEIVLTQSPGTLSLSPGERATLSCRASQSVGSSYLAWYQQKPGQAPRLLIYGAFSRATGIPDRFSGSGSGTDFTLTISRLEPEDFAVYYCQQYGSSPWTFGQGTKVEIKRTVAAPSVFIFPPSDEQLKSGTASVVCLLNNFYPREAKVQWKVDNALQSGNSQESVTEQDSKDSTYSLSSTLTLSKADYEKHKVYACEVTHQGLSSPVTKSFNRGEC

SEQ ID NO: 440 - protein, 262 aa, Artificial Sequence
  Spacer - YV02-2011 LC
QGQSGQGQPCAQMYGYSMCPHTGGGSSGGSISSGLLSGRSDNPGGGSEIVLTQSPGTLSLSPGERATLSCRASQSVGSSYLAWYQQKPGQAPRLLIYGAFSRATGIPDRFSGSGSGTDFTLTISRLEPEDFAVYYCQQYGSSPWTFGQGTKVEIKRTVAAPSVFIFPPSDEQLKSGTASVVCLLNNFYPREAKVQWKVDNALQSGNSQESVTEQDSKDSTYSLSSTLTLSKADYEKHKVYACEVTHQGLSSPVTKSFNRGEC

SEQ ID NO: 441 - protein, 255 aa, Artificial Sequence
  YV02-2011 LC
QPCAQMYGYSMCPHTGGGSSGGSISSGLLSGRSDNPGGGSEIVLTQSPGTLSLSPGERATLSCRASQSVGSSYLAWYQQKPGQAPRLLIYGAFSRATGIPDRFSGSGSGTDFTLTISRLEPEDFAVYYCQQYGSSPWTFGQGTKVEIKRTVAAPSVFIFPPSDEQLKSGTASVVCLLNNFYPREAKVQWKVDNALQSGNSQESVTEQDSKDSTYSLSSTLTLSKADYEKHKVYACEVTHQGLSSPVTKSFNRGEC

SEQ ID NO: 442 - protein, 262 aa, Artificial Sequence
  Spacer - YV03-2011 LC
QGQSGQGLHCRTQMYGYNLCPYGGGSSGGSISSGLLSGRSDNPGGGSEIVLTQSPGTLSLSPGERATLSCRASQSVGSSYLAWYQQKPGQAPRLLIYGAFSRATGIPDRFSGSGSGTDFTLTISRLEPEDFAVYYCQQYGSSPWTFGQGTKVEIKRTVAAPSVFIFPPSDEQLKSGTASVVCLLNNFYPREAKVQWKVDNALQSGNSQESVTEQDSKDSTYSLSSTLTLSKADYEKHKVYACEVTHQGLSSPVTKSFNRGEC

SEQ ID NO: 443 - protein, 255 aa, Artificial Sequence
  YV03-2011 LC
LHCRTQMYGYNLCPYGGGSSGGSISSGLLSGRSDNPGGGSEIVLTQSPGTLSLSPGERATLSCRASQSVGSSYLAWYQQKPGQAPRLLIYGAFSRATGIPDRFSGSGSGTDFTLTISRLEPEDFAVYYCQQYGSSPWTFGQGTKVEIKRTVAAPSVFIFPPSDEQLKSGTASVVCLLNNFYPREAKVQWKVDNALQSGNSQESVTEQDSKDSTYSLSSTLTLSKADYEKHKVYACEVTHQGLSSPVTKSFNRGEC

SEQ ID NO: 444 - protein, 261 aa, Artificial Sequence
  Spacer - YV04-2011 LC
QGQSGSLHCRTQLYGYNLCPYGGGSSGGSISSGLLSGRSDNPGGGSEIVLTQSPGTLSLSPGERATLSCRASQSVGSSYLAWYQQKPGQAPRLLIYGAFSRATGIPDRFSGSGSGTDFTLTISRLEPEDFAVYYCQQYGSSPWTFGQGTKVEIKRTVAAPSVFIFPPSDEQLKSGTASVVCLLNNFYPREAKVQWKVDNALQSGNSQESVTEQDSKDSTYSLSSTLTLSKADYEKHKVYACEVTHQGLSSPVTKSFNRGEC

SEQ ID NO: 445 - protein, 255 aa, Artificial Sequence
  YV04-2011 LC
LHCRTQLYGYNLCPYGGGSSGGSISSGLLSGRSDNPGGGSEIVLTQSPGTLSLSPGERATLSCRASQSVGSSYLAWYQQKPGQAPRLLIYGAFSRATGIPDRFSGSGSGTDFTLTISRLEPEDFAVYYCQQYGSSPWTFGQGTKVEIKRTVAAPSVFIFPPSDEQLKSGTASVVCLLNNFYPREAKVQWKVDNALQSGNSQESVTEQDSKDSTYSLSSTLTLSKADYEKHKVYACEVTHQGLSSPVTKSFNRGEC

SEQ ID NO: 446 - protein, 258 aa, Artificial Sequence
  Spacer - YV23-2011 LC
QGQSGSCLHSLYNVCLDPGGGSSGGSISSGLLSGRSDNPGGGSEIVLTQSPGTLSLSPGERATLSCRASQSVGSSYLAWYQQKPGQAPRLLIYGAFSRATGIPDRFSGSGSGTDFTLTISRLEPEDFAVYYCQQYGSSPWTFGQGTKVEIKRTVAAPSVFIFPPSDEQLKSGTASVVCLLNNFYPREAKVQWKVDNALQSGNSQESVTEQDSKDSTYSLSSTLTLSKADYEKHKVYACEVTHQGLSSPVTKSFNRGEC

SEQ ID NO: 447 - protein, 252 aa, Artificial Sequence
  YV23-2011 LC
CLHSLYNVCLDPGGGSSGGSISSGLLSGRSDNPGGGSEIVLTQSPGTLSLSPGERATLSCRASQSVGSSYLAWYQQKPGQAPRLLIYGAFSRATGIPDRFSGSGSGTDFTLTISRLEPEDFAVYYCQQYGSSPWTFGQGTKVEIKRTVAAPSVFIFPPSDEQLKSGTASVVCLLNNFYPREAKVQWKVDNALQSGNSQESVTEQDSKDSTYSLSSTLTLSKADYEKHKVYACEVTHQGLSSPVTKSFNRGEC

SEQ ID NO: 448 - protein, 259 aa, Artificial Sequence
  Spacer - YV39-2011 LC
QGQSGSCRTQLYGYNLCPYGGGSSGGSISSGLLSGRSDNPGGGSEIVLTQSPGTLSLSPGERATLSCRASQSVGSSYLAWYQQKPGQAPRLLIYGAFSRATGIPDRFSGSGSGTDFTLTISRLEPEDFAVYYCQQYGSSPWTFGQGTKVEIKRTVAAPSVFIFPPSDEQLKSGTASVVCLLNNFYPREAKVQWKVDNALQSGNSQESVTEQDSKDSTYSLSSTLTLSKADYEKHKVYACEVTHQGLSSPVTKSFNRGEC

SEQ ID NO: 449 - protein, 253 aa, Artificial Sequence
  YV39-2011 LC
CRTQLYGYNLCPYGGGSSGGSISSGLLSGRSDNPGGGSEIVLTQSPGTLSLSPGERATLSCRASQSVGSSYLAWYQQKPGQAPRLLIYGAFSRATGIPDRFSGSGSGTDFTLTISRLEPEDFAVYYCQQYGSSPWTFGQGTKVEIKRTVAAPSVFIFPPSDEQLKSGTASVVCLLNNFYPREAKVQWKVDNALQSGNSQESVTEQDSKDSTYSLSSTLTLSKADYEKHKVYACEVTHQGLSSPVTKSFNRGEC

SEQ ID NO: 450 - protein, 261 aa, Artificial Sequence
  Spacer - YV61-2011 LC
QGQSGSYISDCPYHPMCHDYQGGGSSGGSISSGLLSGRSDNPGGGSEIVLTQSPGTLSLSPGERATLSCRASQSVGSSYLAWYQQKPGQAPRLLIYGAFSRATGIPDRFSGSGSGTDFTLTISRLEPEDFAVYYCQQYGSSPWTFGQGTKVEIKRTVAAPSVFIFPPSDEQLKSGTASVVCLLNNFYPREAKVQWKVDNALQSGNSQESVTEQDSKDSTYSLSSTLTLSKADYEKHKVYACEVTHQGLSSPVTKSFNRGEC

SEQ ID NO: 451 - protein, 255 aa, Artificial Sequence
  YV61-2011 LC
YISDCPYHPMCHDYQGGGSSGGSISSGLLSGRSDNPGGGSEIVLTQSPGTLSLSPGERATLSCRASQSVGSSYLAWYQQKPGQAPRLLIYGAFSRATGIPDRFSGSGSGTDFTLTISRLEPEDFAVYYCQQYGSSPWTFGQGTKVEIKRTVAAPSVFIFPPSDEQLKSGTASVVCLLNNFYPREAKVQWKVDNALQSGNSQESVTEQDSKDSTYSLSSTLTLSKADYEKHKVYACEVTHQGLSSPVTKSFNRGEC

SEQ ID NO: 452 - protein, 261 aa, Artificial Sequence
  Spacer - YV62-2011 LC
QGQSGSFRNTCPYHPMCHDYRGGGSSGGSISSGLLSGRSDNPGGGSEIVLTQSPGTLSLSPGERATLSCRASQSVGSSYLAWYQQKPGQAPRLLIYGAFSRATGIPDRFSGSGSGTDFTLTISRLEPEDFAVYYCQQYGSSPWTFGQGTKVEIKRTVAAPSVFIFPPSDEQLKSGTASVVCLLNNFYPREAKVQWKVDNALQSGNSQESVTEQDSKDSTYSLSSTLTLSKADYEKHKVYACEVTHQGLSSPVTKSFNRGEC

SEQ ID NO: 453 - protein, 255 aa, Artificial Sequence
  YV62-2011 LC
FRNTCPYHPMCHDYRGGGSSGGSISSGLLSGRSDNPGGGSEIVLTQSPGTLSLSPGERATLSCRASQSVGSSYLAWYQQKPGQAPRLLIYGAFSRATGIPDRFSGSGSGTDFTLTISRLEPEDFAVYYCQQYGSSPWTFGQGTKVEIKRTVAAPSVFIFPPSDEQLKSGTASVVCLLNNFYPREAKVQWKVDNALQSGNSQESVTEQDSKDSTYSLSSTLTLSKADYEKHKVYACEVTHQGLSSPVTKSFNRGEC

SEQ ID NO: 454 - protein, 261 aa, Artificial Sequence
  Spacer - YV63-2011 LC
QGQSGSRECHMWMFGVNLCPYGGGSSGGSISSGLLSGRSDNPGGGSEIVLTQSPGTLSLSPGERATLSCRASQSVGSSYLAWYQQKPGQAPRLLIYGAFSRATGIPDRFSGSGSGTDFTLTISRLEPEDFAVYYCQQYGSSPWTFGQGTKVEIKRTVAAPSVFIFPPSDEQLKSGTASVVCLLNNFYPREAKVQWKVDNALQSGNSQESVTEQDSKDSTYSLSSTLTLSKADYEKHKVYACEVTHQGLSSPVTKSFNRGEC

SEQ ID NO: 455 - protein, 255 aa, Artificial Sequence
  YV63-2011 LC
RECHMWMFGVNLCPYGGGSSGGSISSGLLSGRSDNPGGGSEIVLTQSPGTLSLSPGERATLSCRASQSVGSSYLAWYQQKPGQAPRLLIYGAFSRATGIPDRFSGSGSGTDFTLTISRLEPEDFAVYYCQQYGSSPWTFGQGTKVEIKRTVAAPSVFIFPPSDEQLKSGTASVVCLLNNFYPREAKVQWKVDNALQSGNSQESVTEQDSKDSTYSLSSTLTLSKADYEKHKVYACEVTHQGLSSPVTKSFNRGEC

SEQ ID NO: 456 - protein, 262 aa, Artificial Sequence
  Spacer - YV64-2011 LC
QGQSGSAVCHMYMYGYNLCPFGGGSSGGSISSGLLSGRSDNPGGGSEIVLTQSPGTLSLSPGERATLSCRASQSVGSSYLAWYQQKPGQAPRLLIYGAFSRATGIPDRFSGSGSGTDFTLTISRLEPEDFAVYYCQQYGSSPWTFGQGTKVEIKRTVAAPSVFIFPPSDEQLKSGTASVVCLLNNFYPREAKVQWKVDNALQSGNSQESVTEQDSKDSTYSLSSTLTLSKADYEKHKVYACEVTHQGLSSPVTKSFNRGECC

SEQ ID NO: 457 - protein, 255 aa, Artificial Sequence
  YV64-2011 LC
AVCHMYMYGYNLCPFGGGSSGGSISSGLLSGRSDNPGGGSEIVLTQSPGTLSLSPGERATLSCRASQSVGSSYLAWYQQKPGQAPRLLIYGAFSRATGIPDRFSGSGSGTDFTLTISRLEPEDFAVYYCQQYGSSPWTFGQGTKVEIKRTVAAPSVFIFPPSDEQLKSGTASVVCLLNNFYPREAKVQWKVDNALQSGNSQESVTEQDSKDSTYSLSSTLTLSKADYEKHKVYACEVTHQGLSSPVTKSFNRGEC

SEQ ID NO: 458 - protein, 262 aa, Artificial Sequence
  Spacer - YV65-2011 LC
QGQSGQGRSCPQMYGYSMCPHTGGGSSGGSISSGLLSGRSDNPGGGSEIVLTQSPGTLSLSPGERATLSCRASQSVGSSYLAWYQQKPGQAPRLLIYGAFSRATGIPDRFSGSGSGTDFTLTISRLEPEDFAVYYCQQYGSSPWTFGQGTKVEIKRTVAAPSVFIFPPSDEQLKSGTASVVCLLNNFYPREAKVQWKVDNALQSGNSQESVTEQDSKDSTYSLSSTLTLSKADYEKHKVYACEVTHQGLSSPVTKSFNRGEC

SEQ ID NO: 459 - protein, 255 aa, Artificial Sequence
  YV65-2011 LC
RSCPQMYGYSMCPHTGGGSSGGSISSGLLSGRSDNPGGGSEIVLTQSPGTLSLSPGERATLSCRASQSVGSSYLAWYQQKPGQAPRLLIYGAFSRATGIPDRFSGSGSGTDFTLTISRLEPEDFAVYYCQQYGSSPWTFGQGTKVEIKRTVAAPSVFIFPPSDEQLKSGTASVVCLLNNFYPREAKVQWKVDNALQSGNSQESVTEQDSKDSTYSLSSTLTLSKADYEKHKVYACEVTHQGLSSPVTKSFNRGEC

SEQ ID NO: 460 - protein, 262 aa, Artificial Sequence
  Spacer - YV66-2011 LC
QGQSGQGQPCAQMFGYSMCPHTGGGSSGGSISSGLLSGRSDNPGGGSEIVLTQSPGTLSLSPGERATLSCRASQSVGSSYLAWYQQKPGQAPRLLIYGAFSRATGIPDRFSGSGSGTDFTLTISRLEPEDFAVYYCQQYGSSPWTFGQGTKVEIKRTVAAPSVFIFPPSDEQLKSGTASVVCLLNNFYPREAKVQWKVDNALQSGNSQESVTEQDSKDSTYSLSSTLTLSKADYEKHKVYACEVTHQGLSSPVTKSFNRGEC

SEQ ID NO: 461 - protein, 255 aa, Artificial Sequence
  YV66-2011 LC
QPCAQMFGYSMCPHTGGGSSGGSISSGLLSGRSDNPGGGSEIVLTQSPGTLSLSPGERATLSCRASQSVGSSYLAWYQQKPGQAPRLLIYGAFSRATGIPDRFSGSGSGTDFTLTISRLEPEDFAVYYCQQYGSSPWTFGQGTKVEIKRTVAAPSVFIFPPSDEQLKSGTASVVCLLNNFYPREAKVQWKVDNALQSGNSQESVTEQDSKDSTYSLSSTLTLSKADYEKHKVYACEVTHQGLSSPVTKSFNRGEC

SEQ ID NO: 462 - protein, 262 aa, Artificial Sequence
  Spacer - YV01-2012 LC
QGQSGQGDFSCLHSMYNVCLDPGGGSSGGSISSGLLSGRSANPGGGSEIVLTQSPGTLSLSPGERATLSCRASQSVGSSYLAWYQQKPGQAPRLLIYGAFSRATGIPDRFSGSGSGTDFTLTISRLEPEDFAVYYCQQYGSSPWTFGQGTKVEIKRTVAAPSVFIFPPSDEQLKSGTASVVCLLNNFYPREAKVQWKVDNALQSGNSQESVTEQDSKDSTYSLSSTLTLSKADYEKHKVYACEVTHQGLSSPVTKSFNRGEC

SEQ ID NO: 463 - protein, 255 aa, Artificial Sequence
  YV01-2012 LC
DFSCLHSMYNVCLDPGGGSSGGSISSGLLSGRSANPGGGSEIVLTQSPGTLSLSPGERATLSCRASQSVGSSYLAWYQQKPGQAPRLLIYGAFSRATGIPDRFSGSGSGTDFTLTISRLEPEDFAVYYCQQYGSSPWTFGQGTKVEIKRTVAAPSVFIFPPSDEQLKSGTASVVCLLNNFYPREAKVQWKVDNALQSGNSQESVTEQDSKDSTYSLSSTLTLSKADYEKHKVYACEVTHQGLSSPVTKSFNRGEC

SEQ ID NO: 464 - protein, 262 aa, Artificial Sequence
  Spacer - YV02-2012 LC
QGQSGQGQPCAQMYGYSMCPHTGGGSSGGSISSGLLSGRSANPGGGSEIVLTQSPGTLSLSPGERATLSCRASQSVGSSYLAWYQQKPGQAPRLLIYGAFSRATGIPDRFSGSGSGTDFTLTISRLEPEDFAVYYCQQYGSSPWTFGQGTKVEIKRTVAAPSVFIFPPSDEQLKSGTASVVCLLNNFYPREAKVQWKVDNALQSGNSQESVTEQDSKDSTYSLSSTLTLSKADYEKHKVYACEVTHQGLSSPVTKSFNRGEC

SEQ ID NO: 465 - protein, 255 aa, Artificial Sequence
  YV02-2012 LC
QPCAQMYGYSMCPHTGGGSSGGSISSGLLSGRSANPGGGSEIVLTQSPGTLSLSPGERATLSCRASQSVGSSYLAWYQQKPGQAPRLLIYGAFSRATGIPDRFSGSGSGTDFTLTISRLEPEDFAVYYCQQYGSSPWTFGQGTKVEIKRTVAAPSVFIFPPSDEQLKSGTASVVCLLNNFYPREAKVQWKVDNALQSGNSQESVTEQDSKDSTYSLSSTLTLSKADYEKHKVYACEVTHQGLSSPVTKSFNRGEC

SEQ ID NO: 466 - protein, 262 aa, Artificial Sequence
  Spacer - YV03-2012 LC
QGQSGQGLHCRTQMYGYNLCPYGGGSSGGSISSGLLSGRSANPGGGSEIVLTQSPGTLSLSPGERATLSCRASQSVGSSYLAWYQQKPGQAPRLLIYGAFSRATGIPDRFSGSGSGTDFTLTISRLEPEDFAVYYCQQYGSSPWTFGQGTKVEIKRTVAAPSVFIFPPSDEQLKSGTASVVCLLNNFYPREAKVQWKVDNALQSGNSQESVTEQDSKDSTYSLSSTLTLSKADYEKHKVYACEVTHQGLSSPVTKSFNRGEC

SEQ ID NO: 467 - protein, 255 aa, Artificial Sequence
  YV03-2012 LC
LHCRTQMYGYNLCPYGGGSSGGSISSGLLSGRSANPGGGSEIVLTQSPGTLSLSPGERATLSCRASQSVGSSYLAWYQQKPGQAPRLLIYGAFSRATGIPDRFSGSGSGTDFTLTISRLEPEDFAVYYCQQYGSSPWTFGQGTKVEIKRTVAAPSVFIFPPSDEQLKSGTASVVCLLNNFYPREAKVQWKVDNALQSGNSQESVTEQDSKDSTYSLSSTLTLSKADYEKHKVYACEVTHQGLSSPVTKSFNRGEC

SEQ ID NO: 468 - protein, 261 aa, Artificial Sequence
  Spacer - YV04-2012 LC
QGQSGSLHCRTQLYGYNLCPYGGGSSGGSISSGLLSGRSANPGGGSEIVLTQSPGTLSLSPGERATLSCRASQSVGSSYLAWYQQKPGQAPRLLIYGAFSRATGIPDRFSGSGSGTDFTLTISRLEPEDFAVYYCQQYGSSPWTFGQGTKVEIKRTVAAPSVFIFPPSDEQLKSGTASVVCLLNNFYPREAKVQWKVDNALQSGNSQESVTEQDSKDSTYSLSSTLTLSKADYEKHKVYACEVTHQGLSSPVTKSFNRGEC

SEQ ID NO: 469 - protein, 255 aa, Artificial Sequence
  YV04-2012 LC
LHCRTQLYGYNLCPYGGGSSGGSISSGLLSGRSANPGGGSEIVLTQSPGTLSLSPGERATLSCRASQSVGSSYLAWYQQKPGQAPRLLIYGAFSRATGIPDRFSGSGSGTDFTLTISRLEPEDFAVYYCQQYGSSPWTFGQGTKVEIKRTVAAPSVFIFPPSDEQLKSGTASVVCLLNNFYPREAKVQWKVDNALQSGNSQESVTEQDSKDSTYSLSSTLTLSKADYEKHKVYACEVTHQGLSSPVTKSFNRGEC

SEQ ID NO: 470 - protein, 258 aa, Artificial Sequence
  Spacer - YV23-2012 LC
QGQSGSCLHSLYNVCLDPGGGSSGGSISSGLLSGRSANPGGGSEIVLTQSPGTLSLSPGERATLSCRASQSVGSSYLAWYQQKPGQAPRLLIYGAFSRATGIPDRFSGSGSGTDFTLTISRLEPEDFAVYYCQQYGSSPWTFGQGTKVEIKRTVAAPSVFIFPPSDEQLKSGTASVVCLLNNFYPREAKVQWKVDNALQSGNSQESVTEQDSKDSTYSLSSTLTLSKADYEKHKVYACEVTHQGLSSPVTKSFNRGEC

SEQ ID NO: 471 - protein, 252 aa, Artificial Sequence
  YV23-2012 LC
CLHSLYNVCLDPGGGSSGGSISSGLLSGRSANPGGGSEIVLTQSPGTLSLSPGERATLSCRASQSVGSSYLAWYQQKPGQAPRLLIYGAFSRATGIPDRFSGSGSGTDFTLTISRLEPEDFAVYYCQQYGSSPWTFGQGTKVEIKRTVAAPSVFIFPPSDEQLKSGTASVVCLLNNFYPREAKVQWKVDNALQSGNSQESVTEQDSKDSTYSLSSTLTLSKADYEKHKVYACEVTHQGLSSPVTKSFNRGEC

SEQ ID NO: 472 - protein, 259 aa, Artificial Sequence
  Spacer - YV39-2012 LC
QGQSGSCRTQLYGYNLCPYGGGSSGGSISSGLLSGRSANPGGGSEIVLTQSPGTLSLSPGERATLSCRASQSVGSSYLAWYQQKPGQAPRLLIYGAFSRATGIPDRFSGSGSGTDFTLTISRLEPEDFAVYYCQQYGSSPWTFGQGTKVEIKRTVAAPSVFIFPPSDEQLKSGTASVVCLLNNFYPREAKVQWKVDNALQSGNSQESVTEQDSKDSTYSLSSTLTLSKADYEKHKVYACEVTHQGLSSPVTKSFNRGEC

SEQ ID NO: 473 - protein, 253 aa, Artificial Sequence
  YV39-2012 LC
CRTQLYGYNLCPYGGGSSGGSISSGLLSGRSANPGGGSEIVLTQSPGTLSLSPGERATLSCRASQSVGSSYLAWYQQKPGQAPRLLIYGAFSRATGIPDRFSGSGSGTDFTLTISRLEPEDFAVYYCQQYGSSPWTFGQGTKVEIKRTVAAPSVFIFPPSDEQLKSGTASVVCLLNNFYPREAKVQWKVDNALQSGNSQESVTEQDSKDSTYSLSSTLTLSKADYEKHKVYACEVTHQGLSSPVTKSFNRGEC

SEQ ID NO: 474 - protein, 261 aa, Artificial Sequence
  Spacer - YV61-2012 LC
QGQSGSYISDCPYHPMCHDYQGGGSSGGSISSGLLSGRSANPGGGSEIVLTQSPGTLSLSPGERATLSCRASQSVGSSYLAWYQQKPGQAPRLLIYGAFSRATGIPDRFSGSGSGTDFTLTISRLEPEDFAVYYCQQYGSSPWTFGQGTKVEIKRTVAAPSVFIFPPSDEQLKSGTASVVCLLNNFYPREAKVQWKVDNALQSGNSQESVTEQDSKDSTYSLSSTLTLSKADYEKHKVYACEVTHQGLSSPVTKSFNRGEC

SEQ ID NO: 475 - protein, 255 aa, Artificial Sequence
  YV61-2012 LC
YISDCPYHPMCHDYQGGGSSGGSISSGLLSGRSANPGGGSEIVLTQSPGTLSLSPGERATLSCRASQSVGSSYLAWYQQKPGQAPRLLIYGAFSRATGIPDRFSGSGSGTDFTLTISRLEPEDFAVYYCQQYGSSPWTFGQGTKVEIKRTVAAPSVFIFPPSDEQLKSGTASVVCLLNNFYPREAKVQWKVDNALQSGNSQESVTEQDSKDSTYSLSSTLTLSKADYEKHKVYACEVTHQGLSSPVTKSFNRGEC

SEQ ID NO: 476 - protein, 261 aa, Artificial Sequence
  Spacer - YV62-2012 LC
QGQSGSFRNTCPYHPMCHDYRGGGSSGGSISSGLLSGRSANPGGGSEIVLTQSPGTLSLSPGERATLSCRASQSVGSSYLAWYQQKPGQAPRLLIYGAFSRATGIPDRFSGSGSGTDFTLTISRLEPEDFAVYYCQQYGSSPWTFGQGTKVEIKRTVAAPSVFIFPPSDEQLKSGTASVVCLLNNFYPREAKVQWKVDNALQSGNSQESVTEQDSKDSTYSLSSTLTLSKADYEKHKVYACEVTHQGLSSPVTKSFNRGEC

SEQ ID NO: 477 - protein, 255 aa, Artificial Sequence
  YV62-2012 LC
FRNTCPYHPMCHDYRGGGSSGGSISSGLLSGRSANPGGGSEIVLTQSPGTLSLSPGERATLSCRASQSVGSSYLAWYQQKPGQAPRLLIYGAFSRATGIPDRFSGSGSGTDFTLTISRLEPEDFAVYYCQQYGSSPWTFGQGTKVEIKRTVAAPSVFIFPPSDEQLKSGTASVVCLLNNFYPREAKVQWKVDNALQSGNSQESVTEQDSKDSTYSLSSTLTLSKADYEKHKVYACEVTHQGLSSPVTKSFNRGEC

SEQ ID NO: 478 - protein, 261 aa, Artificial Sequence
  Spacer - YV63-2012 LC
QGQSGSRECHMWMFGVNLCPYGGGSSGGSISSGLLSGRSANPGGGSEIVLTQSPGTLSLSPGERATLSCRASQSVGSSYLAWYQQKPGQAPRLLIYGAFSRATGIPDRFSGSGSGTDFTLTISRLEPEDFAVYYCQQYGSSPWTFGQGTKVEIKRTVAAPSVFIFPPSDEQLKSGTASVVCLLNNFYPREAKVQWKVDNALQSGNSQESVTEQDSKDSTYSLSSTLTLSKADYEKHKVYACEVTHQGLSSPVTKSFNRGEC

SEQ ID NO: 479 - protein, 255 aa, Artificial Sequence
  YV63-2012 LC
RECHMWMFGVNLCPYGGGSSGGSISSGLLSGRSANPGGGSEIVLTQSPGTLSLSPGERATLSCRASQSVGSSYLAWYQQKPGQAPRLLIYGAFSRATGIPDRFSGSGSGTDFTLTISRLEPEDFAVYYCQQYGSSPWTFGQGTKVEIKRTVAAPSVFIFPPSDEQLKSGTASVVCLLNNFYPREAKVQWKVDNALQSGNSQESVTEQDSKDSTYSLSSTLTLSKADYEKHKVYACEVTHQGLSSPVTKSFNRGEC

SEQ ID NO: 480 - protein, 261 aa, Artificial Sequence
  Spacer - YV64-2012 LC
QGQSGSAVCHMYMYGYNLCPFGGGSSGGSISSGLLSGRSANPGGGSEIVLTQSPGTLSLSPGERATLSCRASQSVGSSYLAWYQQKPGQAPRLLIYGAFSRATGIPDRFSGSGSGTDFTLTISRLEPEDFAVYYCQQYGSSPWTFGQGTKVEIKRTVAAPSVFIFPPSDEQLKSGTASVVCLLNNFYPREAKVQWKVDNALQSGNSQESVTEQDSKDSTYSLSSTLTLSKADYEKHKVYACEVTHQGLSSPVTKSFNRGEC

SEQ ID NO: 481 - protein, 255 aa, Artificial Sequence
  YV64-2012 LC
AVCHMYMYGYNLCPFGGGSSGGSISSGLLSGRSANPGGGSEIVLTQSPGTLSLSPGERATLSCRASQSVGSSYLAWYQQKPGQAPRLLIYGAFSRATGIPDRFSGSGSGTDFTLTISRLEPEDFAVYYCQQYGSSPWTFGQGTKVEIKRTVAAPSVFIFPPSDEQLKSGTASVVCLLNNFYPREAKVQWKVDNALQSGNSQESVTEQDSKDSTYSLSSTLTLSKADYEKHKVYACEVTHQGLSSPVTKSFNRGEC

SEQ ID NO: 482 - protein, 262 aa, Artificial Sequence
  Spacer - YV65-2012 LC
QGQSGQGRSCPQMYGYSMCPHTGGGSSGGSISSGLLSGRSANPGGGSEIVLTQSPGTLSLSPGERATLSCRASQSVGSSYLAWYQQKPGQAPRLLIYGAFSRATGIPDRFSGSGSGTDFTLTISRLEPEDFAVYYCQQYGSSPWTFGQGTKVEIKRTVAAPSVFIFPPSDEQLKSGTASVVCLLNNFYPREAKVQWKVDNALQSGNSQESVTEQDSKDSTYSLSSTLTLSKADYEKHKVYACEVTHQGLSSPVTKSFNRGEC

SEQ ID NO: 483 - protein, 255 aa, Artificial Sequence
  YV65-2012 LC
RSCPQMYGYSMCPHTGGGSSGGSISSGLLSGRSANPGGGSEIVLTQSPGTLSLSPGERATLSCRASQSVGSSYLAWYQQKPGQAPRLLIYGAFSRATGIPDRFSGSGSGTDFTLTISRLEPEDFAVYYCQQYGSSPWTFGQGTKVEIKRTVAAPSVFIFPPSDEQLKSGTASVVCLLNNFYPREAKVQWKVDNALQSGNSQESVTEQDSKDSTYSLSSTLTLSKADYEKHKVYACEVTHQGLSSPVTKSFNRGEC

SEQ ID NO: 484 - protein, 262 aa, Artificial Sequence
  Spacer - YV66-2012 LC
QGQSGQGQPCAQMFGYSMCPHTGGGSSGGSISSGLLSGRSANPGGGSEIVLTQSPGTLSLSPGERATLSCRASQSVGSSYLAWYQQKPGQAPRLLIYGAFSRATGIPDRFSGSGSGTDFTLTISRLEPEDFAVYYCQQYGSSPWTFGQGTKVEIKRTVAAPSVFIFPPSDEQLKSGTASVVCLLNNFYPREAKVQWKVDNALQSGNSQESVTEQDSKDSTYSLSSTLTLSKADYEKHKVYACEVTHQGLSSPVTKSFNRGEC

SEQ ID NO: 485 - protein, 255 aa, Artificial Sequence
  YV66-2012 LC
QPCAQMFGYSMCPHTGGGSSGGSISSGLLSGRSANPGGGSEIVLTQSPGTLSLSPGERATLSCRASQSVGSSYLAWYQQKPGQAPRLLIYGAFSRATGIPDRFSGSGSGTDFTLTISRLEPEDFAVYYCQQYGSSPWTFGQGTKVEIKRTVAAPSVFIFPPSDEQLKSGTASVVCLLNNFYPREAKVQWKVDNALQSGNSQESVTEQDSKDSTYSLSSTLTLSKADYEKHKVYACEVTHQGLSSPVTKSFNRGEC

SEQ ID NO: 486 - protein, 267 aa, Artificial Sequence
  Spacer - YV01-3001 LC
QGQSGQGDFSCLHSMYNVCLDPGGGSSGGSAVGLLAPPGGLSGRSDNHGGGSEIVLTQSPGTLSLSPGERATLSCRASQSVGSSYLAWYQQKPGQAPRLLIYGAFSRATGIPDRFSGSGSGTDFTLTISRLEPEDFAVYYCQQYGSSPWTFGQGTKVEIKRTVAAPSVFIFPPSDEQLKSGTASVVCLLNNFYPREAKVQWKVDNALQSGNSQESVTEQDSKDSTYSLSSTLTLSKADYEKHKVYACEVTHQGLSSPVTKSFNRGEC

SEQ ID NO: 487 - protein, 260 aa, Artificial Sequence
  YV01-3001 LC
DFSCLHSMYNVCLDPGGGSSGGSAVGLLAPPGGLSGRSDNHGGGSEIVLTQSPGTLSLSPGERATLSCRASQSVGSSYLAWYQQKPGQAPRLLIYGAFSRATGIPDRFSGSGSGTDFTLTISRLEPEDFAVYYCQQYGSSPWTFGQGTKVEIKRTVAAPSVFIFPPSDEQLKSGTASVVCLLNNFYPREAKVQWKVDNALQSGNSQESVTEQDSKDSTYSLSSTLTLSKADYEKHKVYACEVTHQGLSSPVTKSFNRGEC

SEQ ID NO: 488 - protein, 267 aa, Artificial Sequence
  Spacer - YV02-3001 LC
QGQSGQGQPCAQMYGYSMCPHTGGGSSGGSAVGLLAPPGGLSGRSDNHGGGSEIVLTQSPGTLSLSPGERATLSCRASQSVGSSYLAWYQQKPGQAPRLLIYGAFSRATGIPDRFSGSGSGTDFTLTISRLEPEDFAVYYCQQYGSSPWTFGQGTKVEIKRTVAAPSVFIFPPSDEQLKSGTASVVCLLNNFYPREAKVQWKVDNALQSGNSQESVTEQDSKDSTYSLSSTLTLSKADYEKHKVYACEVTHQGLSSPVTKSFNRGEC

SEQ ID NO: 489 - protein, 260 aa, Artificial Sequence
  YV02-3001 LC
QPCAQMYGYSMCPHTGGGSSGGSAVGLLAPPGGLSGRSDNHGGGSEIVLTQSPGTLSLSPGERATLSCRASQSVGSSYLAWYQQKPGQAPRLLIYGAFSRATGIPDRFSGSGSGTDFTLTISRLEPEDFAVYYCQQYGSSPWTFGQGTKVEIKRTVAAPSVFIFPPSDEQLKSGTASVVCLLNNFYPREAKVQWKVDNALQSGNSQESVTEQDSKDSTYSLSSTLTLSKADYEKHKVYACEVTHQGLSSPVTKSFNRGEC

SEQ ID NO: 490 - protein, 267 aa, Artificial Sequence
  Spacer - YV03-3001 LC
QGQSGQGLHCRTQMYGYNLCPYGGGSSGGSAVGLLAPPGGLSGRSDNHGGGSEIVLTQSPGTLSLSPGERATLSCRASQSVGSSYLAWYQQKPGQAPRLLIYGAFSRATGIPDRFSGSGSGTDFTLTISRLEPEDFAVYYCQQYGSSPWTFGQGTKVEIKRTVAAPSVFIFPPSDEQLKSGTASVVCLLNNFYPREAKVQWKVDNALQSGNSQESVTEQDSKDSTYSLSSTLTLSKADYEKHKVYACEVTHQGLSSPVTKSFNRGEC

SEQ ID NO: 491 - protein, 260 aa, Artificial Sequence
  YV03-3001 LC
LHCRTQMYGYNLCPYGGGSSGGSAVGLLAPPGGLSGRSDNHGGGSEIVLTQSPGTLSLSPGERATLSCRASQSVGSSYLAWYQQKPGQAPRLLIYGAFSRATGIPDRFSGSGSGTDFTLTISRLEPEDFAVYYCQQYGSSPWTFGQGTKVEIKRTVAAPSVFIFPPSDEQLKSGTASVVCLLNNFYPREAKVQWKVDNALQSGNSQESVTEQDSKDSTYSLSSTLTLSKADYEKHKVYACEVTHQGLSSPVTKSFNRGEC

SEQ ID NO: 492 - protein, 265 aa, Artificial Sequence
  Spacer - YV04-3001 LC
QGQSGSLHCRTQLYGYNLCPYGGGSSGGAVGLLAPPGGLSGRSDNHGGGSEIVLTQSPGTLSLSPGERATLSCRASQSVGSSYLAWYQQKPGQAPRLLIYGAFSRATGIPDRFSGSGSGTDFTLTISRLEPEDFAVYYCQQYGSSPWTFGQGTKVEIKRTVAAPSVFIFPPSDEQLKSGTASVVCLLNNFYPREAKVQWKVDNALQSGNSQESVTEQDSKDSTYSLSSTLTLSKADYEKHKVYACEVTHQGLSSPVTKSFNRGEC

SEQ ID NO: 493 - protein, 259 aa, Artificial Sequence
  YV04-3001 LC
LHCRTQLYGYNLCPYGGGSSGGAVGLLAPPGGLSGRSDNHGGGSEIVLTQSPGTLSLSPGERATLSCRASQSVGSSYLAWYQQKPGQAPRLLIYGAFSRATGIPDRFSGSGSGTDFTLTISRLEPEDFAVYYCQQYGSSPWTFGQGTKVEIKRTVAAPSVFIFPPSDEQLKSGTASVVCLLNNFYPREAKVQWKVDNALQSGNSQESVTEQDSKDSTYSLSSTLTLSKADYEKHKVYACEVTHQGLSSPVTKSFNRGEC

SEQ ID NO: 494 - protein, 260 aa, Artificial Sequence
  Spacer - YV06-3001 LC
QGQSGSCAQMYGYSMCGGGSSGGAVGLLAPPGGLSGRSDNHGGGSEIVLTQSPGTLSLSPGERATLSCRASQSVGSSYLAWYQQKPGQAPRLLIYGAFSRATGIPDRFSGSGSGTDFTLTISRLEPEDFAVYYCQQYGSSPWTFGQGTKVEIKRTVAAPSVFIFPPSDEQLKSGTASVVCLLNNFYPREAKVQWKVDNALQSGNSQESVTEQDSKDSTYSLSSTLTLSKADYEKHKVYACEVTHQGLSSPVTKSFNRGEC

SEQ ID NO: 495 - protein, 254 aa, Artificial Sequence
  YV06-3001 LC
CAQMYGYSMCGGGSSGGAVGLLAPPGGLSGRSDNHGGGSEIVLTQSPGTLSLSPGERATLSCRASQSVGSSYLAWYQQKPGQAPRLLIYGAFSRATGIPDRFSGSGSGTDFTLTISRLEPEDFAVYYCQQYGSSPWTFGQGTKVEIKRTVAAPSVFIFPPSDEQLKSGTASVVCLLNNFYPREAKVQWKVDNALQSGNSQESVTEQDSKDSTYSLSSTLTLSKADYEKHKVYACEVTHQGLSSPVTKSFNRGEC

SEQ ID NO: 496 - protein, 265 aa, Artificial Sequence
  Spacer - YV09-3001 LC
QGQSGSFGTACPNHPMCHDWQGGGSSGGAVGLLAPPGGLSGRSDNHGGGSEIVLTQSPGTLSLSPGERATLSCRASQSVGSSYLAWYQQKPGQAPRLLIYGAFSRATGIPDRFSGSGSGTDFTLTISRLEPEDFAVYYCQQYGSSPWTFGQGTKVEIKRTVAAPSVFIFPPSDEQLKSGTASVVCLLNNFYPREAKVQWKVDNALQSGNSQESVTEQDSKDSTYSLSSTLTLSKADYEKHKVYACEVTHQGLSSPVTKSFNRGEC

SEQ ID NO: 497 - protein, 259 aa, Artificial Sequence
  YV09-3001 LC
FGTACPNHPMCHDWQGGGSSGGAVGLLAPPGGLSGRSDNHGGGSEIVLTQSPGTLSLSPGERATLSCRASQSVGSSYLAWYQQKPGQAPRLLIYGAFSRATGIPDRFSGSGSGTDFTLTISRLEPEDFAVYYCQQYGSSPWTFGQGTKVEIKRTVAAPSVFIFPPSDEQLKSGTASVVCLLNNFYPREAKVQWKVDNALQSGNSQESVTEQDSKDSTYSLSSTLTLSKADYEKHKVYACEVTHQGLSSPVTKSFNRGEC

SEQ ID NO: 498 - protein, 262 aa, Artificial Sequence
  Spacer - YV23-3001 LC
QGQSGSCLHSLYNVCLDPGGGSSGGAVGLLAPPGGLSGRSDNHGGGSEIVLTQSPGTLSLSPGERATLSCRASQSVGSSYLAWYQQKPGQAPRLLIYGAFSRATGIPDRFSGSGSGTDFTLTISRLEPEDFAVYYCQQYGSSPWTFGQGTKVEIKRTVAAPSVFIFPPSDEQLKSGTASVVCLLNNFYPREAKVQWKVDNALQSGNSQESVTEQDSKDSTYSLSSTLTLSKADYEKHKVYACEVTHQGLSSPVTKSFNRGEC

SEQ ID NO: 499 - protein, 256 aa, Artificial Sequence
  YV23-3001 LC
CLHSLYNVCLDPGGGSSGGAVGLLAPPGGLSGRSDNHGGGSEIVLTQSPGTLSLSPGERATLSCRASQSVGSSYLAWYQQKPGQAPRLLIYGAFSRATGIPDRFSGSGSGTDFTLTISRLEPEDFAVYYCQQYGSSPWTFGQGTKVEIKRTVAAPSVFIFPPSDEQLKSGTASVVCLLNNFYPREAKVQWKVDNALQSGNSQESVTEQDSKDSTYSLSSTLTLSKADYEKHKVYACEVTHQGLSSPVTKSFNRGEC

SEQ ID NO: 500 - protein, 262 aa, Artificial Sequence
  Spacer - YV27-3001 LC
QGQSGSQPCAQMYGYSMCGGGSSGGAVGLLAPPGGLSGRSDNHGGGSEIVLTQSPGTLSLSPGERATLSCRASQSVGSSYLAWYQQKPGQAPRLLIYGAFSRATGIPDRFSGSGSGTDFTLTISRLEPEDFAVYYCQQYGSSPWTFGQGTKVEIKRTVAAPSVFIFPPSDEQLKSGTASVVCLLNNFYPREAKVQWKVDNALQSGNSQESVTEQDSKDSTYSLSSTLTLSKADYEKHKVYACEVTHQGLSSPVTKSFNRGEC

SEQ ID NO: 501 - protein, 256 aa, Artificial Sequence
  YV27-3001 LC
QPCAQMYGYSMCGGGSSGGAVGLLAPPGGLSGRSDNHGGGSEIVLTQSPGTLSLSPGERATLSCRASQSVGSSYLAWYQQKPGQAPRLLIYGAFSRATGIPDRFSGSGSGTDFTLTISRLEPEDFAVYYCQQYGSSPWTFGQGTKVEIKRTVAAPSVFIFPPSDEQLKSGTASVVCLLNNFYPREAKVQWKVDNALQSGNSQESVTEQDSKDSTYSLSSTLTLSKADYEKHKVYACEVTHQGLSSPVTKSFNRGEC

SEQ ID NO: 502 - protein, 263 aa, Artificial Sequence
  Spacer - YV29-3001 LC
QGQSGSCAQMYGYSMCAHTGGGSSGGAVGLLAPPGGLSGRSDNHGGGSEIVLTQSPGTLSLSPGERATLSCRASQSVGSSYLAWYQQKPGQAPRLLIYGAFSRATGIPDRFSGSGSGTDFTLTISRLEPEDFAVYYCQQYGSSPWTFGQGTKVEIKRTVAAPSVFIFPPSDEQLKSGTASVVCLLNNFYPREAKVQWKVDNALQSGNSQESVTEQDSKDSTYSLSSTLTLSKADYEKHKVYACEVTHQGLSSPVTKSFNRGEC

SEQ ID NO: 503 - protein, 257 aa, Artificial Sequence
  YV29-3001 LC
CAQMYGYSMCAHTGGGSSGGAVGLLAPPGGLSGRSDNHGGGSEIVLTQSPGTLSLSPGERATLSCRASQSVGSSYLAWYQQKPGQAPRLLIYGAFSRATGIPDRFSGSGSGTDFTLTISRLEPEDFAVYYCQQYGSSPWTFGQGTKVEIKRTVAAPSVFIFPPSDEQLKSGTASVVCLLNNFYPREAKVQWKVDNALQSGNSQESVTEQDSKDSTYSLSSTLTLSKADYEKHKVYACEVTHQGLSSPVTKSFNRGEC

SEQ ID NO: 504 - protein, 261 aa, Artificial Sequence
  Spacer - YV32-3001 LC
QGQSGSCPNHPLCHDWQGGGSSGGAVGLLAPPGGLSGRSDNHGGGSEIVLTQSPGTLSLSPGERATLSCRASQSVGSSYLAWYQQKPGQAPRLLIYGAFSRATGIPDRFSGSGSGTDFTLTISRLEPEDFAVYYCQQYGSSPWTFGQGTKVEIKRTVAAPSVFIFPPSDEQLKSGTASVVCLLNNFYPREAKVQWKVDNALQSGNSQESVTEQDSKDSTYSLSSTLTLSKADYEKHKVYACEVTHQGLSSPVTKSFNRGEC

SEQ ID NO: 505 - protein, 255 aa, Artificial Sequence
  YV32-3001 LC
CPNHPLCHDWQGGGSSGGAVGLLAPPGGLSGRSDNHGGGSEIVLTQSPGTLSLSPGERATLSCRASQSVGSSYLAWYQQKPGQAPRLLIYGAFSRATGIPDRFSGSGSGTDFTLTISRLEPEDFAVYYCQQYGSSPWTFGQGTKVEIKRTVAAPSVFIFPPSDEQLKSGTASVVCLLNNFYPREAKVQWKVDNALQSGNSQESVTEQDSKDSTYSLSSTLTLSKADYEKHKVYACEVTHQGLSSPVTKSFNRGEC

SEQ ID NO: 506 - protein, 261 aa, Artificial Sequence
  Spacer - YV33-3001 LC
QGQSGSCPNHPMCADWQGGGSSGGAVGLLAPPGGLSGRSDNHGGGSEIVLTQSPGTLSLSPGERATLSCRASQSVGSSYLAWYQQKPGQAPRLLIYGAFSRATGIPDRFSGSGSGTDFTLTISRLEPEDFAVYYCQQYGSSPWTFGQGTKVEIKRTVAAPSVFIFPPSDEQLKSGTASVVCLLNNFYPREAKVQWKVDNALQSGNSQESVTEQDSKDSTYSLSSTLTLSKADYEKHKVYACEVTHQGLSSPVTKSFNRGEC

SEQ ID NO: 507 - protein, 255 aa, Artificial Sequence
  Spacer - YV33-3001 LC
CPNHPMCADWQGGGSSGGAVGLLAPPGGLSGRSDNHGGGSEIVLTQSPGTLSLSPGERATLSCRASQSVGSSYLAWYQQKPGQAPRLLIYGAFSRATGIPDRFSGSGSGTDFTLTISRLEPEDFAVYYCQQYGSSPWTFGQGTKVEIKRTVAAPSVFIFPPSDEQLKSGTASVVCLLNNFYPREAKVQWKVDNALQSGNSQESVTEQDSKDSTYSLSSTLTLSKADYEKHKVYACEVTHQGLSSPVTKSFNRGEC

SEQ ID NO: 508 - protein, 261 aa, Artificial Sequence
  Spacer - YV35-3001 LC
QGQSGSCPNHPMCHDAQGGGSSGGAVGLLAPPGGLSGRSDNHGGGSEIVLTQSPGTLSLSPGERATLSCRASQSVGSSYLAWYQQKPGQAPRLLIYGAFSRATGIPDRFSGSGSGTDFTLTISRLEPEDFAVYYCQQYGSSPWTFGQGTKVEIKRTVAAPSVFIFPPSDEQLKSGTASVVCLLNNFYPREAKVQWKVDNALQSGNSQESVTEQDSKDSTYSLSSTLTLSKADYEKHKVYACEVTHQGLSSPVTKSFNRGEC

SEQ ID NO: 509 - protein, 255 aa, Artificial Sequence
  YV35-3001 LC
CPNHPMCHDAQGGGSSGGAVGLLAPPGGLSGRSDNHGGGSEIVLTQSPGTLSLSPGERATLSCRASQSVGSSYLAWYQQKPGQAPRLLIYGAFSRATGIPDRFSGSGSGTDFTLTISRLEPEDFAVYYCQQYGSSPWTFGQGTKVEIKRTVAAPSVFIFPPSDEQLKSGTASVVCLLNNFYPREAKVQWKVDNALQSGNSQESVTEQDSKDSTYSLSSTLTLSKADYEKHKVYACEVTHQGLSSPVTKSFNRGEC

SEQ ID NO: 510 - protein, 263 aa, Artificial Sequence
  Spacer - YV39-3001 LC
QGQSGSCRTQLYGYNLCPYGGGSSGGAVGLLAPPGGLSGRSDNHGGGSEIVLTQSPGTLSLSPGERATLSCRASQSVGSSYLAWYQQKPGQAPRLLIYGAFSRATGIPDRFSGSGSGTDFTLTISRLEPEDFAVYYCQQYGSSPWTFGQGTKVEIKRTVAAPSVFIFPPSDEQLKSGTASVVCLLNNFYPREAKVQWKVDNALQSGNSQESVTEQDSKDSTYSLSSTLTLSKADYEKHKVYACEVTHQGLSSPVTKSFNRGEC

SEQ ID NO: 511 - protein, 257 aa, Artificial Sequence
  YV39-3001 LC
CRTQLYGYNLCPYGGGSSGGAVGLLAPPGGLSGRSDNHGGGSEIVLTQSPGTLSLSPGERATLSCRASQSVGSSYLAWYQQKPGQAPRLLIYGAFSRATGIPDRFSGSGSGTDFTLTISRLEPEDFAVYYCQQYGSSPWTFGQGTKVEIKRTVAAPSVFIFPPSDEQLKSGTASVVCLLNNFYPREAKVQWKVDNALQSGNSQESVTEQDSKDSTYSLSSTLTLSKADYEKHKVYACEVTHQGLSSPVTKSFNRGEC

SEQ ID NO: 512 - protein, 263 aa, Artificial Sequence
  Spacer - YV41-3001 LC
QGQSGSCRTQLYGYNLCPAGGGSSGGAVGLLAPPGGLSGRSDNHGGGSEIVLTQSPGTLSLSPGERATLSCRASQSVGSSYLAWYQQKPGQAPRLLIYGAFSRATGIPDRFSGSGSGTDFTLTISRLEPEDFAVYYCQQYGSSPWTFGQGTKVEIKRTVAAPSVFIFPPSDEQLKSGTASVVCLLNNFYPREAKVQWKVDNALQSGNSQESVTEQDSKDSTYSLSSTLTLSKADYEKHKVYACEVTHQGLSSPVTKSFNRGEC

SEQ ID NO: 513 - protein, 257 aa, Artificial Sequence
  YV41-3001 LC
CRTQLYGYNLCPAGGGSSGGAVGLLAPPGGLSGRSDNHGGGSEIVLTQSPGTLSLSPGERATLSCRASQSVGSSYLAWYQQKPGQAPRLLIYGAFSRATGIPDRFSGSGSGTDFTLTISRLEPEDFAVYYCQQYGSSPWTFGQGTKVEIKRTVAAPSVFIFPPSDEQLKSGTASVVCLLNNFYPREAKVQWKVDNALQSGNSQESVTEQDSKDSTYSLSSTLTLSKADYEKHKVYACEVTHQGLSSPVTKSFNRGEC

SEQ ID NO: 514 - protein, 265 aa, Artificial Sequence
  Spacer - YV51-3001 LC
QGQSGSFGAACPNHPICHDWQGGGSSGGAVGLLAPPGGLSGRSDNHGGGSEIVLTQSPGTLSLSPGERATLSCRASQSVGSSYLAWYQQKPGQAPRLLIYGAFSRATGIPDRFSGSGSGTDFTLTISRLEPEDFAVYYCQQYGSSPWTFGQGTKVEIKRTVAAPSVFIFPPSDEQLKSGTASVVCLLNNFYPREAKVQWKVDNALQSGNSQESVTEQDSKDSTYSLSSTLTLSKADYEKHKVYACEVTHQGLSSPVTKSFNRGEC

SEQ ID NO: 515 - protein, 259 aa, Artificial Sequence
  YV51-3001 LC
FGAACPNHPICHDWQGGGSSGGAVGLLAPPGGLSGRSDNHGGGSEIVLTQSPGTLSLSPGERATLSCRASQSVGSSYLAWYQQKPGQAPRLLIYGAFSRATGIPDRFSGSGSGTDFTLTISRLEPEDFAVYYCQQYGSSPWTFGQGTKVEIKRTVAAPSVFIFPPSDEQLKSGTASVVCLLNNFYPREAKVQWKVDNALQSGNSQESVTEQDSKDSTYSLSSTLTLSKADYEKHKVYACEVTHQGLSSPVTKSFNRGEC

SEQ ID NO: 516 - protein, 265 aa, Artificial Sequence
  Spacer - YV52-3001 LC
QGQSGSFGAACPNHPLCHDWQGGGSSGGAVGLLAPPGGLSGRSDNHGGGSEIVLTQSPGTLSLSPGERATLSCRASQSVGSSYLAWYQQKPGQAPRLLIYGAFSRATGIPDRFSGSGSGTDFTLTISRLEPEDFAVYYCQQYGSSPWTFGQGTKVEIKRTVAAPSVFIFPPSDEQLKSGTASVVCLLNNFYPREAKVQWKVDNALQSGNSQESVTEQDSKDSTYSLSSTLTLSKADYEKHKVYACEVTHQGLSSPVTKSFNRGEC

SEQ ID NO: 517 - protein, 259 aa, Artificial Sequence
  YV52-3001 LC
FGAACPNHPLCHDWQGGGSSGGAVGLLAPPGGLSGRSDNHGGGSEIVLTQSPGTLSLSPGERATLSCRASQSVGSSYLAWYQQKPGQAPRLLIYGAFSRATGIPDRFSGSGSGTDFTLTISRLEPEDFAVYYCQQYGSSPWTFGQGTKVEIKRTVAAPSVFIFPPSDEQLKSGTASVVCLLNNFYPREAKVQWKVDNALQSGNSQESVTEQDSKDSTYSLSSTLTLSKADYEKHKVYACEVTHQGLSSPVTKSFNRGEC

SEQ ID NO: 518 - protein, 265 aa, Artificial Sequence
  Spacer - YV53-3001 LC
QGQSGSFGAACPNHPMCHDAQGGGSSGGAVGLLAPPGGLSGRSDNHGGGSEIVLTQSPGTLSLSPGERATLSCRASQSVGSSYLAWYQQKPGQAPRLLIYGAFSRATGIPDRFSGSGSGTDFTLTISRLEPEDFAVYYCQQYGSSPWTFGQGTKVEIKRTVAAPSVFIFPPSDEQLKSGTASVVCLLNNFYPREAKVQWKVDNALQSGNSQESVTEQDSKDSTYSLSSTLTLSKADYEKHKVYACEVTHQGLSSPVTKSFNRGEC

SEQ ID NO: 519 - protein, 259 aa, Artificial Sequence
  YV53-3001 LC
FGAACPNHPMCHDAQGGGSSGGAVGLLAPPGGLSGRSDNHGGGSEIVLTQSPGTLSLSPGERATLSCRASQSVGSSYLAWYQQKPGQAPRLLIYGAFSRATGIPDRFSGSGSGTDFTLTISRLEPEDFAVYYCQQYGSSPWTFGQGTKVEIKRTVAAPSVFIFPPSDEQLKSGTASVVCLLNNFYPREAKVQWKVDNALQSGNSQESVTEQDSKDSTYSLSSTLTLSKADYEKHKVYACEVTHQGLSSPVTKSFNRGEC

SEQ ID NO: 520 - protein, 262 aa, Artificial Sequence
  Spacer - YV54-3001 LC
QGQSGSCLHSAYNACLDPGGGSSGGAVGLLAPPGGLSGRSDNHGGGSEIVLTQSPGTLSLSPGERATLSCRASQSVGSSYLAWYQQKPGQAPRLLIYGAFSRATGIPDRFSGSGSGTDFTLTISRLEPEDFAVYYCQQYGSSPWTFGQGTKVEIKRTVAAPSVFIFPPSDEQLKSGTASVVCLLNNFYPREAKVQWKVDNALQSGNSQESVTEQDSKDSTYSLSSTLTLSKADYEKHKVYACEVTHQGLSSPVTKSFNRGEC

SEQ ID NO: 521 - protein, 256 aa, Artificial Sequence
  YV54-3001 LC
CLHSAYNACLDPGGGSSGGAVGLLAPPGGLSGRSDNHGGGSEIVLTQSPGTLSLSPGERATLSCRASQSVGSSYLAWYQQKPGQAPRLLIYGAFSRATGIPDRFSGSGSGTDFTLTISRLEPEDFAVYYCQQYGSSPWTFGQGTKVEIKRTVAAPSVFIFPPSDEQLKSGTASVVCLLNNFYPREAKVQWKVDNALQSGNSQESVTEQDSKDSTYSLSSTLTLSKADYEKHKVYACEVTHQGLSSPVTKSFNRGEC

SEQ ID NO: 522 - protein, 262 aa, Artificial Sequence
  Spacer - YV55-3001 LC
QGQSGSCAHSAYNVCLDPGGGSSGGAVGLLAPPGGLSGRSDNHGGGSEIVLTQSPGTLSLSPGERATLSCRASQSVGSSYLAWYQQKPGQAPRLLIYGAFSRATGIPDRFSGSGSGTDFTLTISRLEPEDFAVYYCQQYGSSPWTFGQGTKVEIKRTVAAPSVFIFPPSDEQLKSGTASVVCLLNNFYPREAKVQWKVDNALQSGNSQESVTEQDSKDSTYSLSSTLTLSKADYEKHKVYACEVTHQGLSSPVTKSFNRGEC

SEQ ID NO: 523 - protein, 256 aa, Artificial Sequence
  YV55-3001 LC
CAHSAYNVCLDPGGGSSGGAVGLLAPPGGLSGRSDNHGGGSEIVLTQSPGTLSLSPGERATLSCRASQSVGSSYLAWYQQKPGQAPRLLIYGAFSRATGIPDRFSGSGSGTDFTLTISRLEPEDFAVYYCQQYGSSPWTFGQGTKVEIKRTVAAPSVFIFPPSDEQLKSGTASVVCLLNNFYPREAKVQWKVDNALQSGNSQESVTEQDSKDSTYSLSSTLTLSKADYEKHKVYACEVTHQGLSSPVTKSFNRGEC

SEQ ID NO: 524 - protein, 262 aa, Artificial Sequence
  Spacer - YV56-3001 LC
QGQSGSCLHSAYNVCADPGGGSSGGAVGLLAPPGGLSGRSDNHGGGSEIVLTQSPGTLSLSPGERATLSCRASQSVGSSYLAWYQQKPGQAPRLLIYGAFSRATGIPDRFSGSGSGTDFTLTISRLEPEDFAVYYCQQYGSSPWTFGQGTKVEIKRTVAAPSVFIFPPSDEQLKSGTASVVCLLNNFYPREAKVQWKVDNALQSGNSQESVTEQDSKDSTYSLSSTLTLSKADYEKHKVYACEVTHQGLSSPVTKSFNRGEC

SEQ ID NO: 525 - protein, 256 aa, Artificial Sequence
  YV56-3001 LC
CLHSAYNVCADPGGGSSGGAVGLLAPPGGLSGRSDNHGGGSEIVLTQSPGTLSLSPGERATLSCRASQSVGSSYLAWYQQKPGQAPRLLIYGAFSRATGIPDRFSGSGSGTDFTLTISRLEPEDFAVYYCQQYGSSPWTFGQGTKVEIKRTVAAPSVFIFPPSDEQLKSGTASVVCLLNNFYPREAKVQWKVDNALQSGNSQESVTEQDSKDSTYSLSSTLTLSKADYEKHKVYACEVTHQGLSSPVTKSFNRGEC

SEQ ID NO: 526 - protein, 262 aa, Artificial Sequence
  Spacer - YV57-3001 LC
QGQSGSCLHSAYNVCLAPGGGSSGGAVGLLAPPGGLSGRSDNHGGGSEIVLTQSPGTLSLSPGERATLSCRASQSVGSSYLAWYQQKPGQAPRLLIYGAFSRATGIPDRFSGSGSGTDFTLTISRLEPEDFAVYYCQQYGSSPWTFGQGTKVEIKRTVAAPSVFIFPPSDEQLKSGTASVVCLLNNFYPREAKVQWKVDNALQSGNSQESVTEQDSKDSTYSLSSTLTLSKADYEKHKVYACEVTHQGLSSPVTKSFNRGEC

SEQ ID NO: 527 - protein, 256 aa, Artificial Sequence
  YV57-3001 LC
CLHSAYNVCLAPGGGSSGGAVGLLAPPGGLSGRSDNHGGGSEIVLTQSPGTLSLSPGERATLSCRASQSVGSSYLAWYQQKPGQAPRLLIYGAFSRATGIPDRFSGSGSGTDFTLTISRLEPEDFAVYYCQQYGSSPWTFGQGTKVEIKRTVAAPSVFIFPPSDEQLKSGTASVVCLLNNFYPREAKVQWKVDNALQSGNSQESVTEQDSKDSTYSLSSTLTLSKADYEKHKVYACEVTHQGLSSPVTKSFNRGEC

SEQ ID NO: 528 - protein, 262 aa, Artificial Sequence
  Spacer - YV58-3001 LC
QGQSGSCLHSAYNVCLDAGGGSSGGAVGLLAPPGGLSGRSDNHGGGSEIVLTQSPGTLSLSPGERATLSCRASQSVGSSYLAWYQQKPGQAPRLLIYGAFSRATGIPDRFSGSGSGTDFTLTISRLEPEDFAVYYCQQYGSSPWTFGQGTKVEIKRTVAAPSVFIFPPSDEQLKSGTASVVCLLNNFYPREAKVQWKVDNALQSGNSQESVTEQDSKDSTYSLSSTLTLSKADYEKHKVYACEVTHQGLSSPVTKSFNRGEC

SEQ ID NO: 529 - protein, 256 aa, Artificial Sequence
  YV58-3001 LC
CLHSAYNVCLDAGGGSSGGAVGLLAPPGGLSGRSDNHGGGSEIVLTQSPGTLSLSPGERATLSCRASQSVGSSYLAWYQQKPGQAPRLLIYGAFSRATGIPDRFSGSGSGTDFTLTISRLEPEDFAVYYCQQYGSSPWTFGQGTKVEIKRTVAAPSVFIFPPSDEQLKSGTASVVCLLNNFYPREAKVQWKVDNALQSGNSQESVTEQDSKDSTYSLSSTLTLSKADYEKHKVYACEVTHQGLSSPVTKSFNRGEC

SEQ ID NO: 530 - protein, 259 aa, Artificial Sequence
  Spacer - YV39-NSUB LC
QGQSGSCRTQLYGYNLCPYGGGSSGGSGGSGGSGGGSGGGSGGSEIVLTQSPGTLSLSPGERATLSCRASQSVGSSYLAWYQQKPGQAPRLLIYGAFSRATGIPDRFSGSGSGTDFTLTISRLEPEDFAVYYCQQYGSSPWTFGQGTKVEIKRTVAAPSVFIFPPSDEQLKSGTASVVCLLNNFYPREAKVQWKVDNALQSGNSQESVTEQDSKDSTYSLSSTLTLSKADYEKHKVYACEVTHQGLSSPVTKSFNRGEC

SEQ ID NO: 531 - protein, 253 aa, Artificial Sequence
  YV39-NSUB LC
CRTQLYGYNLCPYGGGSSGGSGGSGGSGGGSGGGSGGSEIVLTQSPGTLSLSPGERATLSCRASQSVGSSYLAWYQQKPGQAPRLLIYGAFSRATGIPDRFSGSGSGTDFTLTISRLEPEDFAVYYCQQYGSSPWTFGQGTKVEIKRTVAAPSVFIFPPSDEQLKSGTASVVCLLNNFYPREAKVQWKVDNALQSGNSQESVTEQDSKDSTYSLSSTLTLSKADYEKHKVYACEVTHQGLSSPVTKSFNRGEC

SEQ ID NO: 532 - protein, 2 aa, Artificial Sequence
  Linkers
  MISC_FEATURE (1)..(2): sequence may be repeated any number of times
GS

SEQ ID NO: 533 - protein, 3 aa, Artificial Sequence
  Linkers
  MISC_FEATURE (1)..(3): sequence may be repeated any number of times
GGS

SEQ ID NO: 534 - protein, 5 aa, Artificial Sequence
  Linkers
  MISC_FEATURE (1)..(5): sequence may be repeated any number of times
GSGGS

SEQ ID NO: 535 - protein, 4 aa, Artificial Sequence
  Linkers
  MISC_FEATURE (1)..(4): sequence may be repeated any number of times
GGGS

SEQ ID NO: 536 - protein, 4 aa, Artificial Sequence
  Linkers
GGSG

SEQ ID NO: 537 - protein, 5 aa, Artificial Sequence
  Linkers
GGSGG

SEQ ID NO: 538 - protein, 5 aa, Artificial Sequence
  Linkers
GSGSG

SEQ ID NO: 539 - protein, 5 aa, Artificial Sequence
  Linkers
GSGGG

SEQ ID NO: 540 - protein, 5 aa, Artificial Sequence
  Linkers
GGGSG

SEQ ID NO: 541 - protein, 5 aa, Artificial Sequence
  Linkers
GSSSG

SEQ ID NO: 542 - protein, 8 aa, Artificial Sequence
  Linkers
GGGSSGGS

SEQ ID NO: 543 - protein, 4 aa, Artificial Sequence
  Linkers
GGGS

SEQ ID NO: 544 - protein, 7 aa, Artificial Sequence
  Spacer
QGQSGQG

SEQ ID NO: 545 - protein, 6 aa, Artificial Sequence
  Spacer
GQSGQG

SEQ ID NO: 546 - protein, 6 aa, Artificial Sequence
  Spacer
QGQSGS

SEQ ID NO: 547 - protein, 6 aa, Artificial Sequence
  Spacer
QGQSGQ

SEQ ID NO: 548 - protein, 5 aa, Artificial Sequence
  Spacer
QSGQG

SEQ ID NO: 549 - protein, 5 aa, Artificial Sequence
  Spacer
GQSGS

SEQ ID NO: 550 - protein, 5 aa, Artificial Sequence
  Spacer
QGQSG

SEQ ID NO: 551 - protein, 4 aa, Artificial Sequence
  Spacer
SGQG

SEQ ID NO: 552 - protein, 4 aa, Artificial Sequence
  Spacer
QSGS

SEQ ID NO: 553 - protein, 4 aa, Artificial Sequence
  Spacer
QGQS

SEQ ID NO: 554 - protein, 15 aa, Artificial Sequence
  Consensus Sequence
  MISC_FEATURE (1)..(2): Xaa can be any amino acid
  MISC_FEATURE (4)..(6): Xaa can be any amino acid
XXCXXXMYGYNLCPY

SEQ ID NO: 555 - protein, 15 aa, Artificial Sequence
  Consensus Sequence
  MISC_FEATURE (1)..(3): Xaa can be any amino acid
  MISC_FEATURE (5)..(5): Xaa can be any amino acid
XXXCXHSMYNVCLDP

SEQ ID NO: 556 - protein, 19 aa, Artificial Sequence
  Spacer-YV39
QGQSGSCRTQLYGYNLCPY

SEQ ID NO: 557 - protein, 5 aa, Artificial Sequence
  CDR1 HC for Ipilimumab
SYTMH

SEQ ID NO: 558 - protein, 17 aa, Artificial Sequence
  CDR2 HC for Ipilimumab
FISYDGNNKYYADSVKG

SEQ ID NO: 559 - protein, 9 aa, Artificial Sequence
  CDR3 HC for Ipilimumab
TGWLGPFDY

SEQ ID NO: 560 - protein, 12 aa, Artificial Sequence
  CDR1 LC for Ipilimumab
RASQSVGSSYLA

SEQ ID NO: 561 - protein, 7 aa, Artificial Sequence
  CDR2 LC for Ipilimumab
GAFSRAT

SEQ ID NO: 562 - protein, 9 aa, Artificial Sequence
  CDR3 LC for Ipilimumab
QQYGSSPWT

SEQ ID NO: 563 - protein, 146 aa, Artificial Sequence
  YV39-2001 VL
CRTQLYGYNLCPYGGGSSGGSISSGLLSGRSDNHGGGSEIVLTQSPGTLSLSPGERATLSCRASQSVGSSYLAWYQQKPGQAPRLLIYGAFSRATGIPDRFSGSGSGTDFTLTISRLEPEDFAVYYCQQYGSSPWTFGQGTKVEIK

SEQ ID NO: 564 - protein, 146 aa, Artificial Sequence
  YV39-2011 VL
CRTQLYGYNLCPYGGGSSGGSISSGLLSGRSDNPGGGSEIVLTQSPGTLSLSPGERATLSCRASQSVGSSYLAWYQQKPGQAPRLLIYGAFSRATGIPDRFSGSGSGTDFTLTISRLEPEDFAVYYCQQYGSSPWTFGQGTKVEIK

SEQ ID NO: 565 - protein, 146 aa, Artificial Sequence
  YV39-2012 VL
CRTQLYGYNLCPYGGGSSGGSISSGLLSGRSANPGGGSEIVLTQSPGTLSLSPGERATLSCRASQSVGSSYLAWYQQKPGQAPRLLIYGAFSRATGIPDRFSGSGSGTDFTLTISRLEPEDFAVYYCQQYGSSPWTFGQGTKVEIK

SEQ ID NO: 566 - protein, 12 aa, Artificial Sequence
  MM Consensus Sequence 1
  MISC_FEATURE (2)..(2): Xaa can be L, M, V or T
  MISC_FEATURE (4)..(4): Xaa can be S, V or I
  MISC_FEATURE (5)..(5): Xaa can be F, L, M or A
  MISC_FEATURE (6)..(6): Xaa can be Y or F
  MISC_FEATURE (8)..(8): Xaa can be V or I
CXYXXXNXCLDP

SEQ ID NO: 567 - protein, 13 aa, Artificial Sequence
  MM Consensus Sequence 2
  MISC_FEATURE (11)..(11): Xaa can be P or A
  MISC_FEATURE (12)..(12): Xaa can be H, R or A
CAQMYGYSMCXXT

SEQ ID NO: 568 - protein, 13 aa, Artificial Sequence
  MM Consensus Sequence 3
  MISC_FEATURE (2)..(2): Xaa can be any amino acid
  MISC_FEATURE (3)..(3): Xaa can be M, I, Y, L, N or F
  MISC_FEATURE (4)..(4): Xaa can be Y, W, F, Q or T
  MISC_FEATURE (5)..(5): Xaa can be M or Y
  MISC_FEATURE (8)..(8): Xaa can be Y, V or F
  MISC_FEATURE (9)..(9): Xaa can be N or D
  MISC_FEATURE (13)..(13): Xaa can be Y or F
CXXXXYGXXLCPX

SEQ ID NO: 569 - protein, 12 aa, Artificial Sequence
  MM Consensus Sequence 4
  MISC_FEATURE (1)..(1): Xaa can be N or T
  MISC_FEATURE (2)..(2): Xaa can be S, T, M or A
  MISC_FEATURE (5)..(5): Xaa can be N or Y
  MISC_FEATURE (8)..(8): Xaa can be M or L
  MISC_FEATURE (10)..(10): Xaa can be H, F or Y
  MISC_FEATURE (12)..(12): Xaa can be Y, F or W
XXCPXHPXCXDX

SEQ ID NO: 570 - protein, 14 aa, Artificial Sequence
  Protease Resistant Linker
GGSGGSGGGSGGGS